European Patent Application EP 4 446 410 A2, published October 16, 2024. Title: COMPOSITIONS COMPRISING POLYPEPTIDES HAVING GALACTANASE ACTIVITY AND POLYPEPTIDES HAVING BETA-GALACTOSIDASE ACTIVITY. Applicant: Novozymes A/S. Application EP. The sequence listing filed with the application follows.

SEQUENCE LISTING (85 sequences)

SEQ ID NO: 1 - DNA, 1047 bp, Cohnella sp-60555
  sig_peptide 1..96
  mat_peptide 97..1044
  source 1..1047: mol_type = genomic DNA
  CDS 1..1044
atgatgttcaagagaacggtaacgggcatgatggccttgctgctggtgctggctctgttcgtcgcgcaaggttcgcagccgcaccaagccgccgcggcgccgtcgttcgccaaaggggcggacatcagctgggtgccgggaatggaagcccaggggtacaagtggaaggacaagaacggcgtgcagcgggacattttggacattttgaaaaacgattatcagatcaactccgtgcgcatccgcgtgtgggtcaacccttcgagcagctacacgaacgggtacctgaacaaggaccgtgcggccgcgctggcgaagcgggccaaggcggcggggatgagcgtcatgctgacgctccattacagcgacagctgggcggaccccggccaacagacgaagccggcggcatggaagagctacacgttccagcaactgatggacgccgtgtggaactggacacgcgacgtcatgacgacgatgcaggcgaacggcgtgacgccggactgggtgcagatcggcaacgagacgaacaacggcatgctgtgggacgacggcaaggcttcgctcagcatgaagaattatgcgtggctcgtgaacacgggcaacaacgcggtgaagtcgatcagcagctcgaccaagacgatcgtgcacctggccaacggctacgacaattcgctgttcgtctggaacatcggaggcttgatcgccaacggagcgacgttcgacatcatcggcatgtcgctctatccgagcgcgtcggattggtcggccaaggtgacgcagacgatcgcgaacgcgaacgacatgatctcgcgttacggcaagccgatcatggtgacggagatcggcatggactacagccagccgagcgcggccaagagcttcgtgtcggacatcaagacgaagatccgcaacctgtccggcggcaaggggcaaggcgtgttctactgggagcccgaagcgacgcccggctacaacggcggctacagcatgggcgcctggcaagcggacatgaagccgacgatcgcgctcgagggcttctggaactaa

SEQ ID NO: 2 - protein, 348 aa, Cohnella sp-60555
MMFKRTVTGMMALLLVLALFVAQGSQPHQAAAAPSFAKGADISWVPGMEAQGYKWKDKNGVQRDILDILKNDYQINSVRIRVWVNPSSSYTNGYLNKDRAAALAKRAKAAGMSVMLTLHYSDSWADPGQQTKPAAWKSYTFQQLMDAVWNWTRDVMTTMQANGVTPDWVQIGNETNNGMLWDDGKASLSMKNYAWLVNTGNNAVKSISSSTKTIVHLANGYDNSLFVWNIGGLIANGATFDIIGMSLYPSASDWSAKVTQTIANANDMISRYGKPIMVTEIGMDYSQPSAAKSFVSDIKTKIRNLSGGKGQGVFYWEPEATPGYNGGYSMGAWQADMKPTIALEGFWN

SEQ ID NO: 3 - protein, 316 aa, Cohnella sp-60555
  REGION 1..316: note = mat_peptide
APSFAKGADISWVPGMEAQGYKWKDKNGVQRDILDILKNDYQINSVRIRVWVNPSSSYTNGYLNKDRAAALAKRAKAAGMSVMLTLHYSDSWADPGQQTKPAAWKSYTFQQLMDAVWNWTRDVMTTMQANGVTPDWVQIGNETNNGMLWDDGKASLSMKNYAWLVNTGNNAVKSISSSTKTIVHLANGYDNSLFVWNIGGLIANGATFDIIGMSLYPSASDWSAKVTQTIANANDMISRYGKPIMVTEIGMDYSQPSAAKSFVSDIKTKIRNLSGGKGQGVFYWEPEATPGYNGGYSMGAWQADMKPTIALEGFWN

SEQ ID NO: 4 - protein, 324 aa, synthetic construct
  REGION 1..324: note = Mature sequence with His-tag
  REGION 1..324: note = mat_peptide
HHHHHHPRAPSFAKGADISWVPGMEAQGYKWKDKNGVQRDILDILKNDYQINSVRIRVWVNPSSSYTNGYLNKDRAAALAKRAKAAGMSVMLTLHYSDSWADPGQQTKPAAWKSYTFQQLMDAVWNWTRDVMTTMQANGVTPDWVQIGNETNNGMLWDDGKASLSMKNYAWLVNTGNNAVKSISSSTKTIVHLANGYDNSLFVWNIGGLIANGATFDIIGMSLYPSASDWSAKVTQTIANANDMISRYGKPIMVTEIGMDYSQPSAAKSFVSDIKTKIRNLSGGKGQGVFYWEPEATPGYNGGYSMGAWQADMKPTIALEGFWN

SEQ ID NO: 5 - DNA, 1044 bp, Cohnella xylanilytica
  sig_peptide 1..87
  mat_peptide 88..1041
  source 1..1044: mol_type = genomic DNA
  CDS 1..1041
atgttgcgcaaagcggttgcggtgttcatcaccttggtgttgggactgactctactatcggcgcagggaggacgaccgcaggaagcggcggcggctccgtcgttcgctaagggagcggacatcagctgggtgccgggaatggaagcgcaagggtacaggtggaaggacaagaacggcgtgcagcgggacatcctggacattctcaagaacgattaccagatcaactccgtccgcattcgggtatgggtcaatccttcgagcagctatacgaacggctacctgaacaaggaccgggcggccgcgctcgcgaagcgggcgaaggcggcggggctcagcgtcatgctgacgctgcattacagcgacagctgggccgaccccgggaagcagacgaagccggcggcgtgggccgggtacaacttccagcagctgatggacgcggtgtggaactggacgcgcgaggtcatgacgacgatgcaggccagcggggtgacgccggactgggtgcagatcggcaacgagacgaacaacggcatgctgtgggacgacgggaaggcctcgctgagcatgaagaattacgcctggctcgtcaacacgggcaacaacgcggtcaagtcgatcagcagcgggacgaaaacgatcgtgcatctcgccaacgggtacgacaattcgttgttcgtctggaacatcggcggcctgatcgcgaacggcgccacgttcgacattatcggcatgtcgctgtatccgagcgcgtccgactggtcctcgaaggtgacgcagacgatctccaacgcgaacgatatgatctcccggtacggcaagccgatcatgatcacggagatcggcatggactacaaccagccgtcggcggccaagagcttcgtcgcggatatcaagacgaagatccgcagcctgtccggcggccgagggctcggcgtcttctactgggagccggaggcgaccccgggttataacggaggctataacaagggagcctggcaggcagacatgaagccgacgatcgctctcgaaggttttctgaactaa

SEQ ID NO: 6 - protein, 347 aa, Cohnella xylanilytica
MLRKAVAVFITLVLGLTLLSAQGGRPQEAAAAPSFAKGADISWVPGMEAQGYRWKDKNGVQRDILDILKNDYQINSVRIRVWVNPSSSYTNGYLNKDRAAALAKRAKAAGLSVMLTLHYSDSWADPGKQTKPAAWAGYNFQQLMDAVWNWTREVMTTMQASGVTPDWVQIGNETNNGMLWDDGKASLSMKNYAWLVNTGNNAVKSISSGTKTIVHLANGYDNSLFVWNIGGLIANGATFDIIGMSLYPSASDWSSKVTQTISNANDMISRYGKPIMITEIGMDYNQPSAAKSFVADIKTKIRSLSGGRGLGVFYWEPEATPGYNGGYNKGAWQADMKPTIALEGFLN

SEQ ID NO: 7 - protein, 318 aa, Cohnella xylanilytica
  REGION 1..318: note = mat_peptide
AAAPSFAKGADISWVPGMEAQGYRWKDKNGVQRDILDILKNDYQINSVRIRVWVNPSSSYTNGYLNKDRAAALAKRAKAAGLSVMLTLHYSDSWADPGKQTKPAAWAGYNFQQLMDAVWNWTREVMTTMQASGVTPDWVQIGNETNNGMLWDDGKASLSMKNYAWLVNTGNNAVKSISSGTKTIVHLANGYDNSLFVWNIGGLIANGATFDIIGMSLYPSASDWSSKVTQTISNANDMISRYGKPIMITEIGMDYNQPSAAKSFVADIKTKIRSLSGGRGLGVFYWEPEATPGYNGGYNKGAWQADMKPTIALEGFLN

SEQ ID NO: 8 - protein, 326 aa, synthetic construct
  REGION 1..326: note = Mature sequence with His-tag
  REGION 1..326: note = mat_peptide
HHHHHHPRAAAPSFAKGADISWVPGMEAQGYRWKDKNGVQRDILDILKNDYQINSVRIRVWVNPSSSYTNGYLNKDRAAALAKRAKAAGLSVMLTLHYSDSWADPGKQTKPAAWAGYNFQQLMDAVWNWTREVMTTMQASGVTPDWVQIGNETNNGMLWDDGKASLSMKNYAWLVNTGNNAVKSISSGTKTIVHLANGYDNSLFVWNIGGLIANGATFDIIGMSLYPSASDWSSKVTQTISNANDMISRYGKPIMITEIGMDYNQPSAAKSFVADIKTKIRSLSGGRGLGVFYWEPEATPGYNGGYNKGAWQADMKPTIALEGFLN

SEQ ID NO: 9 - DNA, 1050 bp, Paenibacillus tundrae
  sig_peptide 1..99
  mat_peptide 100..1047
  source 1..1050: mol_type = genomic DNA
  CDS 1..1047
atgttcaaaaatgtaaggggtttcaagacatccatcatgttggcttttgttttgttattcacctccatcatgttgcccgcaggtcagcatgccagcgcagcaccaagtttcgccaaaggagccgacatcagctgggttcccggaatggaagcccaaggttacaaatggaaagataaaaacggggtacagcgtgacatcattgatattttgaaaaaggactatcaaattaactccgttcgcattcgggtctttgttaatccttcgaatgattatgggaacggttacatgaataaggaacgtgcggctacactcgcacaacgtgctaaaaatgccggcatgagcgtaatgcttaccctgcattacagcgactcttgggcagaccctggtcaacagaccaaaccagctgcctggaaaaactataccttccaacagctcatggacgcagtgtggaatcacacacgtgatgtcatgactgcgatgcaaagcaaaggcgttaccccggactgggtacagatcgggaatgaaacaagtaacggcatgttatgggaagatggtaaagcatccaccaacatgaaaaactatgcgtggctggtgaacacaggccataatgcagtgaaatccctgagcagtggcaccaaaaccattgtgcacctggcaggtggggatgataacgccctctatgtatggaatattggtggtttgatcaataatggagctaactttgacatgattgccatgtccctctacccttcggcttccggctggaacacagctgtgacgaatacggtaaacaatgccaaggatatgatcaaccgttatggcaaagagatcatcatctccgaaattggcatggataataaccaggctgcagcaggtaaaagttttgttgcggcgatgaaaaaccaaatccgcaatctgccgaatggcaaaggaaaaggcgtattctactgggagcctcaggctacaccaggttataacagtggctacggcaaaggcgcttggcaatcgaatatgatgccgacagttgtcatggaaggatttattgactag

SEQ ID NO: 10 - protein, 349 aa, Paenibacillus tundrae
MFKNVRGFKTSIMLAFVLLFTSIMLPAGQHASAAPSFAKGADISWVPGMEAQGYKWKDKNGVQRDIIDILKKDYQINSVRIRVFVNPSNDYGNGYMNKERAATLAQRAKNAGMSVMLTLHYSDSWADPGQQTKPAAWKNYTFQQLMDAVWNHTRDVMTAMQSKGVTPDWVQIGNETSNGMLWEDGKASTNMKNYAWLVNTGHNAVKSLSSGTKTIVHLAGGDDNALYVWNIGGLINNGANFDMIAMSLYPSASGWNTAVTNTVNNAKDMINRYGKEIIISEIGMDNNQAAAGKSFVAAMKNQIRNLPNGKGKGVFYWEPQATPGYNSGYGKGAWQSNMMPTVVMEGFID

SEQ ID NO: 11 - protein, 316 aa, Paenibacillus tundrae
  REGION 1..316: note = mat_peptide
APSFAKGADISWVPGMEAQGYKWKDKNGVQRDIIDILKKDYQINSVRIRVFVNPSNDYGNGYMNKERAATLAQRAKNAGMSVMLTLHYSDSWADPGQQTKPAAWKNYTFQQLMDAVWNHTRDVMTAMQSKGVTPDWVQIGNETSNGMLWEDGKASTNMKNYAWLVNTGHNAVKSLSSGTKTIVHLAGGDDNALYVWNIGGLINNGANFDMIAMSLYPSASGWNTAVTNTVNNAKDMINRYGKEIIISEIGMDNNQAAAGKSFVAAMKNQIRNLPNGKGKGVFYWEPQATPGYNSGYGKGAWQSNMMPTVVMEGFID

SEQ ID NO: 12 - protein, 324 aa, synthetic construct
  REGION 1..324: note = Mature sequence with His-tag
  REGION 1..324: note = mat_peptide
HHHHHHPRAPSFAKGADISWVPGMEAQGYKWKDKNGVQRDIIDILKKDYQINSVRIRVFVNPSNDYGNGYMNKERAATLAQRAKNAGMSVMLTLHYSDSWADPGQQTKPAAWKNYTFQQLMDAVWNHTRDVMTAMQSKGVTPDWVQIGNETSNGMLWEDGKASTNMKNYAWLVNTGHNAVKSLSSGTKTIVHLAGGDDNALYVWNIGGLINNGANFDMIAMSLYPSASGWNTAVTNTVNNAKDMINRYGKEIIISEIGMDNNQAAAGKSFVAAMKNQIRNLPNGKGKGVFYWEPQATPGYNSGYGKGAWQSNMMPTVVMEGFID

SEQ ID NO: 13 - DNA, 1056 bp, Paenibacillus barcinonensis
  sig_peptide 1..105
  mat_peptide 106..1053
  source 1..1056: mol_type = genomic DNA
  CDS 1..1053
atgtttaaaaatgtaaggggtttcaaggttaagacaagcgttctgctggcattggttttgttatttacttctattctgctgcctgcaggccagcacgccagcgccgcaccgagctttgccaagggagctgacatcagctgggttcccggcatggaggctcaagggtacaaatggaaggataaaaacggggtacaacgtgatattattgatattttgaaaaaggattaccaaattaactccgttcgtattcgggtattcgttaatccatcgaacgattatggtaacggttacatgaataaggatcgcgcggctgctcttgcacagcgtgccaaaaatgcaggcatgagtgtcatgctcacacttcactacagcgattcctgggcagacccaggcaaacaaagcaaaccagcggcatggaaaaattactccttccaacagctcatggacgctgtctggaattatacacgtgaagtgatgacagctatgcaaaacaaaggggttacgccggactgggtacagatcggtaacgaaacaagcaacggcatgttatgggatgacgggaaagcctctgttaacatgaaaaactatgcatggctcgtgaacacaggacataatgcggtaaaatccattagcagcggcaccaaaacgatcgttcatctggccggtggcgacgacaatgcgctgtatgtctggaatattggcggcctgatcaacaacggcgctaactttgacatgatcgctatgtcgctttacccttccgcttccggctggaatactgcggtgaccaacacggtcaacaatgcaaaggatatgatcaatcggtacggcaaagagatcatgatctccgaaattggcatggacaacaatcaggcggcggcaggcaaaagcttcgtagctgcgatgaaaaatcaaattcgcaatctgccaaatggcaaaggaaaaggcgtattctactgggagccgcaggctacacctggctataacggtggatacggtaaaggcgcttggcagtccaacatgatgccaacagccgtcatggaagggtttattgactaa

SEQ ID NO: 14 - protein, 351 aa, Paenibacillus barcinonensis
MFKNVRGFKVKTSVLLALVLLFTSILLPAGQHASAAPSFAKGADISWVPGMEAQGYKWKDKNGVQRDIIDILKKDYQINSVRIRVFVNPSNDYGNGYMNKDRAAALAQRAKNAGMSVMLTLHYSDSWADPGKQSKPAAWKNYSFQQLMDAVWNYTREVMTAMQNKGVTPDWVQIGNETSNGMLWDDGKASVNMKNYAWLVNTGHNAVKSISSGTKTIVHLAGGDDNALYVWNIGGLINNGANFDMIAMSLYPSASGWNTAVTNTVNNAKDMINRYGKEIMISEIGMDNNQAAAGKSFVAAMKNQIRNLPNGKGKGVFYWEPQATPGYNGGYGKGAWQSNMMPTAVMEGFID

SEQ ID NO: 15 - protein, 316 aa, Paenibacillus barcinonensis
APSFAKGADISWVPGMEAQGYKWKDKNGVQRDIIDILKKDYQINSVRIRVFVNPSNDYGNGYMNKDRAAALAQRAKNAGMSVMLTLHYSDSWADPGKQSKPAAWKNYSFQQLMDAVWNYTREVMTAMQNKGVTPDWVQIGNETSNGMLWDDGKASVNMKNYAWLVNTGHNAVKSISSGTKTIVHLAGGDDNALYVWNIGGLINNGANFDMIAMSLYPSASGWNTAVTNTVNNAKDMINRYGKEIMISEIGMDNNQAAAGKSFVAAMKNQIRNLPNGKGKGVFYWEPQATPGYNGGYGKGAWQSNMMPTAVMEGFID

SEQ ID NO: 16 - protein, 324 aa, synthetic construct
  REGION 1..324: note = Mature sequence with His-tag
  REGION 1..324: note = mat_peptide
HHHHHHPRAPSFAKGADISWVPGMEAQGYKWKDKNGVQRDIIDILKKDYQINSVRIRVFVNPSNDYGNGYMNKDRAAALAQRAKNAGMSVMLTLHYSDSWADPGKQSKPAAWKNYSFQQLMDAVWNYTREVMTAMQNKGVTPDWVQIGNETSNGMLWDDGKASVNMKNYAWLVNTGHNAVKSISSGTKTIVHLAGGDDNALYVWNIGGLINNGANFDMIAMSLYPSASGWNTAVTNTVNNAKDMINRYGKEIMISEIGMDNNQAAAGKSFVAAMKNQIRNLPNGKGKGVFYWEPQATPGYNGGYGKGAWQSNMMPTAVMEGFID

SEQ ID NO: 17 - DNA, 1044 bp, Paenibacillus sp-62603
  sig_peptide 1..93
  mat_peptide 94..1041
  source 1..1044: mol_type = genomic DNA
  CDS 1..1041
atgaaacgaaggttttacagtttgacgcttgttgtcgccttgttaatgactatttttggagtgaatgggggatctgtgccgcaggtcagcgcagctcctgcattcgcgaaaggtgcggacattagctgggtagtcggcatggaggcgcaagggtatacgtggaaggacaaaaacggcgtaactagggacattattcaaattttgaagcaggattaccaaatcaactccgtacgtattcgagtattcgtcaatccttcttcgaactatggcaacgggtatatgaataaagatcgcgctgcaaccttggcgaagcgggcgaaggatgctgggatgagcgtcatgcttacattgcattacagcgattcgtgggcggaccccggaaaacagacaaagccagcggcttgggcaagctattcgttccagcagctgatggatgcagtttataatcatacgcgtgaggtaatgacagctatgcaaagcaaaggtgtcacaccggattgggtgcaaatcggcaacgaaacgaacgatggcatgctctggaatgacgggaaagcttccttaaacatgcaaaactacgcttggctgatcaacactggcaacaatgcggtcaagtccattagttcagctacaaaaacgattgtccacttgtccaacggttatgacaacagtttatttgtctggaatatcggcggactgatcgctaacggagcgaccttcgatattatcgggatgtcactttatcctaccagtgctgattggtcgactaaggttacgcaaacggtcagcaactccaacaatatgatatcgcgttatggcaagccggttatgattaccgaaattggtatggattataaccagcctgccgctgccaaaagctttgtcgctgatataaagacaaaaatacgtaatattgcaggtggaaaagggcttggcgtgttttattgggaaccggaagcgacccctggttataacggaggttataataagggagcttggcaggcggacggcaaaccaacaattgcgcttgacggcttcttgaattaa

SEQ ID NO: 18 - protein, 347 aa, Paenibacillus sp-62603
MKRRFYSLTLVVALLMTIFGVNGGSVPQVSAAPAFAKGADISWVVGMEAQGYTWKDKNGVTRDIIQILKQDYQINSVRIRVFVNPSSNYGNGYMNKDRAATLAKRAKDAGMSVMLTLHYSDSWADPGKQTKPAAWASYSFQQLMDAVYNHTREVMTAMQSKGVTPDWVQIGNETNDGMLWNDGKASLNMQNYAWLINTGNNAVKSISSATKTIVHLSNGYDNSLFVWNIGGLIANGATFDIIGMSLYPTSADWSTKVTQTVSNSNNMISRYGKPVMITEIGMDYNQPAAAKSFVADIKTKIRNIAGGKGLGVFYWEPEATPGYNGGYNKGAWQADGKPTIALDGFLN

SEQ ID NO: 19 - protein, 316 aa, Paenibacillus sp-62603
  REGION 1..316: note = mat_peptide
APAFAKGADISWVVGMEAQGYTWKDKNGVTRDIIQILKQDYQINSVRIRVFVNPSSNYGNGYMNKDRAATLAKRAKDAGMSVMLTLHYSDSWADPGKQTKPAAWASYSFQQLMDAVYNHTREVMTAMQSKGVTPDWVQIGNETNDGMLWNDGKASLNMQNYAWLINTGNNAVKSISSATKTIVHLSNGYDNSLFVWNIGGLIANGATFDIIGMSLYPTSADWSTKVTQTVSNSNNMISRYGKPVMITEIGMDYNQPAAAKSFVADIKTKIRNIAGGKGLGVFYWEPEATPGYNGGYNKGAWQADGKPTIALDGFLN

SEQ ID NO: 20 - protein, 324 aa, synthetic construct
  REGION 1..324: note = Mature sequence with His-tag
  REGION 1..324: note = mat_peptide
HHHHHHPRAPAFAKGADISWVVGMEAQGYTWKDKNGVTRDIIQILKQDYQINSVRIRVFVNPSSNYGNGYMNKDRAATLAKRAKDAGMSVMLTLHYSDSWADPGKQTKPAAWASYSFQQLMDAVYNHTREVMTAMQSKGVTPDWVQIGNETNDGMLWNDGKASLNMQNYAWLINTGNNAVKSISSATKTIVHLSNGYDNSLFVWNIGGLIANGATFDIIGMSLYPTSADWSTKVTQTVSNSNNMISRYGKPVMITEIGMDYNQPAAAKSFVADIKTKIRNIAGGKGLGVFYWEPEATPGYNGGYNKGAWQADGKPTIALDGFLN

SEQ ID NO: 21 - DNA, 1050 bp, Paenibacillus xylanilyticus
  sig_peptide 1..99
  mat_peptide 100..1047
  source 1..1050: mol_type = genomic DNA
  CDS 1..1047
atgcttaaatttgtaaggggttacaaaacatcgattgctcttgttcttgtgttgttgttcacctccattatgctgcctgtgggtcagcatgtcagcgcagcacccagcttcgccaagggggctgatataagctgggtaccaggcatggaagcgcaagggtacaaatggaaagacaaaaatggtgtacagcgtgacattattgatattttgaaaaacgattatcagatcaactcggttcgtatccgggtgtttgttaatccttctaatgattacggcaacgggtacatgaataaggatcgtgtcgctgctttggcacagcgggccaaaaacgcgggcatgagcgtcatgttgactctgcactacagtgattcctgggcagaccctggccaacagaccaaaccggcagcctggaaaaactacaccttccagcagctgatggatgccgtttggaatcatacacgcgatgtgatgacggccatgcagagtaaaggggttacgcctgactgggtacaaatcgggaacgaaacaagcaacggcatgttatgggaggacggtaaagcgtccacgaacatgaaaaattacgcatggctggtgaacacgggccataatgccgtcaagtccatgagtacagggaccaaaacgattgtccatcttgcaggcggtgacgacaatgccctttatgtatggaatatcggcggactgatcaacaacggtgccaacttcgatatgattgccatgtccctctatccttcggcttccggctggaatacagctgtcaccaatacggtgaataatgccaaggacttgatcaaccgctacggcaaagagattatcgtctcagaaatcggcatggacaacaatcagcccgcagctggcaaaagtttcgttgctgcgatgaaaaatcaattccgcaacctgccaaatgggaaaggaaaaggcgtattctactgggagccgcaggctacaccaggttataacggtggttacggcaaaggcgcttggcagtcgaatatgatgccaacagcggtcatggaaggatttatagactag

SEQ ID NO: 22 - protein, 349 aa, Paenibacillus xylanilyticus
MLKFVRGYKTSIALVLVLLFTSIMLPVGQHVSAAPSFAKGADISWVPGMEAQGYKWKDKNGVQRDIIDILKNDYQINSVRIRVFVNPSNDYGNGYMNKDRVAALAQRAKNAGMSVMLTLHYSDSWADPGQQTKPAAWKNYTFQQLMDAVWNHTRDVMTAMQSKGVTPDWVQIGNETSNGMLWEDGKASTNMKNYAWLVNTGHNAVKSMSTGTKTIVHLAGGDDNALYVWNIGGLINNGANFDMIAMSLYPSASGWNTAVTNTVNNAKDLINRYGKEIIVSEIGMDNNQPAAGKSFVAAMKNQFRNLPNGKGKGVFYWEPQATPGYNGGYGKGAWQSNMMPTAVMEGFID

SEQ ID NO: 23 - protein, 316 aa, Paenibacillus xylanilyticus
  REGION 1..316: note = mat_peptide
APSFAKGADISWVPGMEAQGYKWKDKNGVQRDIIDILKNDYQINSVRIRVFVNPSNDYGNGYMNKDRVAALAQRAKNAGMSVMLTLHYSDSWADPGQQTKPAAWKNYTFQQLMDAVWNHTRDVMTAMQSKGVTPDWVQIGNETSNGMLWEDGKASTNMKNYAWLVNTGHNAVKSMSTGTKTIVHLAGGDDNALYVWNIGGLINNGANFDMIAMSLYPSASGWNTAVTNTVNNAKDLINRYGKEIIVSEIGMDNNQPAAGKSFVAAMKNQFRNLPNGKGKGVFYWEPQATPGYNGGYGKGAWQSNMMPTAVMEGFID

SEQ ID NO: 24 - protein, 324 aa, synthetic construct
  REGION 1..324: note = Mature sequence with His-tag
  REGION 1..324: note = mat_peptide
HHHHHHPRAPSFAKGADISWVPGMEAQGYKWKDKNGVQRDIIDILKNDYQINSVRIRVFVNPSNDYGNGYMNKDRVAALAQRAKNAGMSVMLTLHYSDSWADPGQQTKPAAWKNYTFQQLMDAVWNHTRDVMTAMQSKGVTPDWVQIGNETSNGMLWEDGKASTNMKNYAWLVNTGHNAVKSMSTGTKTIVHLAGGDDNALYVWNIGGLINNGANFDMIAMSLYPSASGWNTAVTNTVNNAKDLINRYGKEIIVSEIGMDNNQPAAGKSFVAAMKNQFRNLPNGKGKGVFYWEPQATPGYNGGYGKGAWQSNMMPTAVMEGFID

SEQ ID NO: 25 - DNA, 1638 bp, Paenibacillus sp-18179
  misc_feature 1..3: note = The gene has an alternative start codon gtg which would normally code for Val but is translated to Met when it is the first codon.
  sig_peptide 1..87
  mat_peptide 88..1635
  source 1..1638: mol_type = genomic DNA
  CDS 1..1635
gtgggtaaatgggttagagctattgctttagcaggtgtagttgcactttttacatctatgatcactcctcttcaagaaacaaaggctgctggaggcttcgttatggggggagacgtttcaatgctccatgaagttgagcagttaggcgggaagttttacgatcagggcactccaaaggatgctttgcaaattttaagcgcacatggcatgaatgctgtccgattgcgtctatgggttgacccgtatgacagtttcggaaatccttatggcggtggaacaaacgatctggctacgactatatctcttgcacagcgagcgaaggcacaaggtatggaggtgctgctggattttcacttcagtgatttctgggcagacccagggaagcagaacaagcctaaagcttggcagagcttaacgtacaaccagctgcttactacggtatatgattatacgcatagtgtaattacgcaaatgaaagcggctggcgtgatgcctgatatggttcaggtaggaaacgaggcaagcagcggcatcctctggaatgatggcaaggtggggggaggcattgatgattttacgaaactcggagaactgtttacctctgctattaatgggattaatgcggccctcagctctagtgagaacattgagattgttctgcatttggatcatggcggcgacaacaatttatacacttggtggttcgataaaattgaagcggagaacgtggattacgatattatcggcttgacctactatccgttttggcatggaacgatgggagaattggcgtataatcttaatgcgatcagcagtcgttacaataaggacgtaatgattgtggaaacgtcgtatggctttacgctggatgatggtgatggtttaggcaactctttttacacggcggaagaaagcattgggggttacccggctacagtagaaggccagacggcgtatttgcgggatttgaaggaaattgttagggatgtcccaaacaaccgcggccgcggcattttctggtgggagccgacatggctgcctgttgcaggggctaactgggggacggatgcaggcaagctgtacaacaatgatactggactactatctaatccttgggacaatcagaccttgtttgattttaatggaaatgtgttgtctacagtttcagtatttacacaaagtgctccaaccaaccttgttgctaatcatagctttgaggccgatggttggacaacaacaccatctagctggaatcgctgggcagccgatacggcatcctataatgctattaaggttgaagaaaacggtattacgggcagctataagctgacgcattggagtgattctgcttatgaggcctctacgtaccagactgtttcaggattaagcaatggtacctatactttatccgcttgggtgcttaacagtggcggacaaaatacgctgcagctttacgctaaaaattacgggggttcagaacggaacgtcaatcttcctgttagcccaacaaagtgggtaaaagtaaaaattgaaaacatcagtgttacaaatggtcaaatcgaattaggcatttattcagatgcgaatgctgataattggatgaacctcgataacgtcaaactttataaaacaaactag

SEQ ID NO: 26 - protein, 545 aa, Paenibacillus sp-18179
VGKWVRAIALAGVVALFTSMITPLQETKAAGGFVMGGDVSMLHEVEQLGGKFYDQGTPKDALQILSAHGMNAVRLRLWVDPYDSFGNPYGGGTNDLATTISLAQRAKAQGMEVLLDFHFSDFWADPGKQNKPKAWQSLTYNQLLTTVYDYTHSVITQMKAAGVMPDMVQVGNEASSGILWNDGKVGGGIDDFTKLGELFTSAINGINAALSSSENIEIVLHLDHGGDNNLYTWWFDKIEAENVDYDIIGLTYYPFWHGTMGELAYNLNAISSRYNKDVMIVETSYGFTLDDGDGLGNSFYTAEESIGGYPATVEGQTAYLRDLKEIVRDVPNNRGRGIFWWEPTWLPVAGANWGTDAGKLYNNDTGLLSNPWDNQTLFDFNGNVLSTVSVFTQSAPTNLVANHSFEADGWTTTPSSWNRWAADTASYNAIKVEENGITGSYKLTHWSDSAYEASTYQTVSGLSNGTYTLSAWVLNSGGQNTLQLYAKNYGGSERNVNLPVSPTKWVKVKIENISVTNGQIELGIYSDANADNWMNLDNVKLYKTN

SEQ ID NO: 27 - protein, 516 aa, Paenibacillus sp-18179
  REGION 1..516: note = mat_peptide
AGGFVMGGDVSMLHEVEQLGGKFYDQGTPKDALQILSAHGMNAVRLRLWVDPYDSFGNPYGGGTNDLATTISLAQRAKAQGMEVLLDFHFSDFWADPGKQNKPKAWQSLTYNQLLTTVYDYTHSVITQMKAAGVMPDMVQVGNEASSGILWNDGKVGGGIDDFTKLGELFTSAINGINAALSSSENIEIVLHLDHGGDNNLYTWWFDKIEAENVDYDIIGLTYYPFWHGTMGELAYNLNAISSRYNKDVMIVETSYGFTLDDGDGLGNSFYTAEESIGGYPATVEGQTAYLRDLKEIVRDVPNNRGRGIFWWEPTWLPVAGANWGTDAGKLYNNDTGLLSNPWDNQTLFDFNGNVLSTVSVFTQSAPTNLVANHSFEADGWTTTPSSWNRWAADTASYNAIKVEENGITGSYKLTHWSDSAYEASTYQTVSGLSNGTYTLSAWVLNSGGQNTLQLYAKNYGGSERNVNLPVSPTKWVKVKIENISVTNGQIELGIYSDANADNWMNLDNVKLYKTN

SEQ ID NO: 28 - protein, 524 aa, synthetic construct
  REGION 1..524: note = Mature sequence with His-tag
  REGION 1..524: note = mat_peptide
HHHHHHPRAGGFVMGGDVSMLHEVEQLGGKFYDQGTPKDALQILSAHGMNAVRLRLWVDPYDSFGNPYGGGTNDLATTISLAQRAKAQGMEVLLDFHFSDFWADPGKQNKPKAWQSLTYNQLLTTVYDYTHSVITQMKAAGVMPDMVQVGNEASSGILWNDGKVGGGIDDFTKLGELFTSAINGINAALSSSENIEIVLHLDHGGDNNLYTWWFDKIEAENVDYDIIGLTYYPFWHGTMGELAYNLNAISSRYNKDVMIVETSYGFTLDDGDGLGNSFYTAEESIGGYPATVEGQTAYLRDLKEIVRDVPNNRGRGIFWWEPTWLPVAGANWGTDAGKLYNNDTGLLSNPWDNQTLFDFNGNVLSTVSVFTQSAPTNLVANHSFEADGWTTTPSSWNRWAADTASYNAIKVEENGITGSYKLTHWSDSAYEASTYQTVSGLSNGTYTLSAWVLNSGGQNTLQLYAKNYGGSERNVNLPVSPTKWVKVKIENISVTNGQIELGIYSDANADNWMNLDNVKLYKTN

SEQ ID NO: 29 - DNA, 1053 bp, Paenibacillus peoriae
  sig_peptide 1..99
  mat_peptide 100..1050
  source 1..1053: mol_type = genomic DNA
  CDS 1..1050
atgaaaacaggtaaccgcacgatggtatttgcgatgttgatcttgctttccagcttattgtatccgttcggctctgtagggttgggtgcggcttcggccgcccctgctttcgccaaaggagcagatataagctgggtagcaggaatggaagcgcaaggtatgacttggaaggataaaaagggtgttcgtcgagatatactgcaaattttgcgagatgactatcagatcaactcggtacgtatccgtgtgtgggtaaaccccgacatgaaagattatgcaagcggatacatgaatgccgaaaaggcagcagaactggcgcagcgagctaaaaaattgggtatgagcgttatgctgactctacattatagtgattcctgggcagatccagggcaacagaacaaaccttatgcgtggcgcaattttacatttacacaactcatggatgcagtctggtctcatacggtttatgttatgaacacgatgaaaagcaagggggtaacaccggactgggtgcagatcggtaatgagacgaacaatggaatgctctgggaagacggcaaagcttcggtgaacatgaaaaactatgcctggctcgtcaatacaggtaataatgctgtaaaatcggtaagcagcagtactaaaacgatagtacatttagccaacggggataacggttccgtgttgaactggaatatcggcggactgattgataatggagctcagtttgatctcatcgggctgtctctgtatccgtctccttctgactggcagggcaaggtggatcagacgattacgaatgccaataacctcattgccaaatacggtaaaggtattgtcatcagtgaaatcgggatggaatataacgaacctgcagcttccaaggcatttatttctgcaatcaaaacaaaggttcggaacatgggaggcggcaaaggcacaggggtattttattgggagccggctgcaactccaggttacaatcaaggttataacaaaggtgcttggcaggctgacggtaaaccaacctcagctttggagggatttgtaaattaa

SEQ ID NO: 30 - protein, 350 aa, Paenibacillus peoriae
MKTGNRTMVFAMLILLSSLLYPFGSVGLGAASAAPAFAKGADISWVAGMEAQGMTWKDKKGVRRDILQILRDDYQINSVRIRVWVNPDMKDYASGYMNAEKAAELAQRAKKLGMSVMLTLHYSDSWADPGQQNKPYAWRNFTFTQLMDAVWSHTVYVMNTMKSKGVTPDWVQIGNETNNGMLWEDGKASVNMKNYAWLVNTGNNAVKSVSSSTKTIVHLANGDNGSVLNWNIGGLIDNGAQFDLIGLSLYPSPSDWQGKVDQTITNANNLIAKYGKGIVISEIGMEYNEPAASKAFISAIKTKVRNMGGGKGTGVFYWEPAATPGYNQGYNKGAWQADGKPTSALEGFVN

SEQ ID NO: 31 - protein, 317 aa, Paenibacillus peoriae
  REGION 1..317: note = mat_peptide
APAFAKGADISWVAGMEAQGMTWKDKKGVRRDILQILRDDYQINSVRIRVWVNPDMKDYASGYMNAEKAAELAQRAKKLGMSVMLTLHYSDSWADPGQQNKPYAWRNFTFTQLMDAVWSHTVYVMNTMKSKGVTPDWVQIGNETNNGMLWEDGKASVNMKNYAWLVNTGNNAVKSVSSSTKTIVHLANGDNGSVLNWNIGGLIDNGAQFDLIGLSLYPSPSDWQGKVDQTITNANNLIAKYGKGIVISEIGMEYNEPAASKAFISAIKTKVRNMGGGKGTGVFYWEPAATPGYNQGYNKGAWQADGKPTSALEGFVN

SEQ ID NO: 32 - protein, 325 aa, synthetic construct
  REGION 1..325: note = Mature sequence with His-tag
  REGION 1..325: note = mat_peptide
HHHHHHPRAPAFAKGADISWVAGMEAQGMTWKDKKGVRRDILQILRDDYQINSVRIRVWVNPDMKDYASGYMNAEKAAELAQRAKKLGMSVMLTLHYSDSWADPGQQNKPYAWRNFTFTQLMDAVWSHTVYVMNTMKSKGVTPDWVQIGNETNNGMLWEDGKASVNMKNYAWLVNTGNNAVKSVSSSTKTIVHLANGDNGSVLNWNIGGLIDNGAQFDLIGLSLYPSPSDWQGKVDQTITNANNLIAKYGKGIVISEIGMEYNEPAASKAFISAIKTKVRNMGGGKGTGVFYWEPAATPGYNQGYNKGAWQADGKPTSALEGFVN

SEQ ID NO: 33 - DNA, 1050 bp, Paenibacillus xylanexedens
  sig_peptide 1..99
  mat_peptide 100..1047
  source 1..1050: mol_type = genomic DNA
  CDS 1..1047
atgttcaaaaatgtaaggggtttcaggatatccatcatgttggcttttgttttgttattcacctccatcatgttgcccgcaggtcagcatgccagcgcagcaccaagtttcgccaaaggagccgacatcagttgggttcccggaatggaagctcaaggctacaaatggaaagataaaaacggggtacagcgtgacatcattgatattttgaaaaatgactatcaaatcaattccgttcgtattcgggtctttgttaatccttcgaacgattatgggaacggttacatgaacaaggatcgtgcggctgcactcgcacaacgtgccaagaatgccggcatgagcgtaatgctcaccctgcactacagcgattcctgggcagaccctggtcaacagaccaaaccagctgcctggaaaaactacacgttccagcagctcatggatgcggtgtggaatcacacacgtgatgtcatgactgcaatgcaaagcaaaggcgttaccccggactgggtacagatcgggaatgaaacaagcaacggcatgttatgggaagatggcaaagcatctaccaacatgaaaaactatgcgtggctggtaaacacaggccataatgcagtgaaatccctgagcagcggcaccaaaaccattgtgcatctggcaggtggagatgataacgccctctatgtatggaatattggaggcctgatcaataacggagccaactttgacatgattgcgatgtccctctacccttcggcttccggctggaacacagctgtgacgaatacagtaaacaatgccaaggatatgatcaaccgttatggcaaagagatcattatctccgaaattggtatggacaataaccaggctgcagctggtaaaagttttgttgcggcgatgaaaaaccaaatccgcaatctgccgaatggtaaaggcaaaggcgtattctactgggagcctcaggctacaccaggatacaacagcggctatggcaaaggtgcatggcaatcgaatatgatgccgacggtagtcatggaaggatttattgactag

SEQ ID NO: 34 - protein, 349 aa, Paenibacillus xylanexedens
MFKNVRGFRISIMLAFVLLFTSIMLPAGQHASAAPSFAKGADISWVPGMEAQGYKWKDKNGVQRDIIDILKNDYQINSVRIRVFVNPSNDYGNGYMNKDRAAALAQRAKNAGMSVMLTLHYSDSWADPGQQTKPAAWKNYTFQQLMDAVWNHTRDVMTAMQSKGVTPDWVQIGNETSNGMLWEDGKASTNMKNYAWLVNTGHNAVKSLSSGTKTIVHLAGGDDNALYVWNIGGLINNGANFDMIAMSLYPSASGWNTAVTNTVNNAKDMINRYGKEIIISEIGMDNNQAAAGKSFVAAMKNQIRNLPNGKGKGVFYWEPQATPGYNSGYGKGAWQSNMMPTVVMEGFID

SEQ ID NO: 35 - protein, 316 aa, Paenibacillus xylanexedens
  REGION 1..316: note = mat_peptide
APSFAKGADISWVPGMEAQGYKWKDKNGVQRDIIDILKNDYQINSVRIRVFVNPSNDYGNGYMNKDRAAALAQRAKNAGMSVMLTLHYSDSWADPGQQTKPAAWKNYTFQQLMDAVWNHTRDVMTAMQSKGVTPDWVQIGNETSNGMLWEDGKASTNMKNYAWLVNTGHNAVKSLSSGTKTIVHLAGGDDNALYVWNIGGLINNGANFDMIAMSLYPSASGWNTAVTNTVNNAKDMINRYGKEIIISEIGMDNNQAAAGKSFVAAMKNQIRNLPNGKGKGVFYWEPQATPGYNSGYGKGAWQSNMMPTVVMEGFID

SEQ ID NO: 36 - protein, 324 aa, synthetic construct
  REGION 1..324: note = Mature sequence with His-tag
  REGION 1..324: note = mat_peptide
HHHHHHPRAPSFAKGADISWVPGMEAQGYKWKDKNGVQRDIIDILKNDYQINSVRIRVFVNPSNDYGNGYMNKDRAAALAQRAKNAGMSVMLTLHYSDSWADPGQQTKPAAWKNYTFQQLMDAVWNHTRDVMTAMQSKGVTPDWVQIGNETSNGMLWEDGKASTNMKNYAWLVNTGHNAVKSLSSGTKTIVHLAGGDDNALYVWNIGGLINNGANFDMIAMSLYPSASGWNTAVTNTVNNAKDMINRYGKEIIISEIGMDNNQAAAGKSFVAAMKNQIRNLPNGKGKGVFYWEPQATPGYNSGYGKGAWQSNMMPTVVMEGFID

SEQ ID NO: 37 - DNA, 1044 bp, Cohnella laeviribosi
  sig_peptide 1..93
  mat_peptide 94..1041
  source 1..1044: mol_type = genomic DNA
  CDS 1..1041
atgaaaagaaaaacgttcggatggctgttgacggcgctgctcggtttgaccctggcgctcggcaacgccgtgtctcccggcgacgcgaaagccgccccggcatttgcgaaaggcgcggacatcagctgggttccgggcatggaggcgcaagggtacaaatggaaggacaaaaacggcgtgcagcgggacatcattgatattttaaagcaggattaccagatcaactccgtccggatccgcgtgtttgtcaatccgtcaagcgattacggcaacggctacttgaacaaggaacgcgcggccgacttggcccagcgggcgaaaaacgccggcatgagcgtcatgctgacgctgcactacagcgattcgtgggcggaccccggcaagcaaaccaagccggccgcgtggcaaaattatacgttcgagcaattgatggacgccgtatggaactggacgcgcgatgtgatgacgacgatgcagagcagaggcgttacgccggactgggtgcagatcggcaacgagacgaacaacggcatgctgtgggatgacggcaaggcgtccgtcaacatgcgtaattacgcctggctcgtcaataccggcaacaatgcggtcaagtcgatcagcagctccacgaagacgatcgtccatctttccaacggctacgacaattcgctgttcgtctggaacatcggtgggctgatcagcaacggcgcgacgtttgacattatcggcatgtcgctgtacccgtccgcgtccgactggcagacgaaggtcaatcagacgatcagcaacgcgaacgatctgatttcgcgctacggcaagagcatcatgatctccgaaatcggcatggactacaaccagccttcggccgcgaagagcttcatctccgacatcaagacgaaggtccggaatctttccggaggcaaagggcttggcgtgttttattgggagcccgaggctacccccggctacaacggcggctacaacaagggcgcctggcagtccgacatgaagccgacgatcgcgctggaaggcttcctgaactga

SEQ ID NO: 38 - protein, 347 aa, Cohnella laeviribosi
MKRKTFGWLLTALLGLTLALGNAVSPGDAKAAPAFAKGADISWVPGMEAQGYKWKDKNGVQRDIIDILKQDYQINSVRIRVFVNPSSDYGNGYLNKERAADLAQRAKNAGMSVMLTLHYSDSWADPGKQTKPAAWQNYTFEQLMDAVWNWTRDVMTTMQSRGVTPDWVQIGNETNNGMLWDDGKASVNMRNYAWLVNTGNNAVKSISSSTKTIVHLSNGYDNSLFVWNIGGLISNGATFDIIGMSLYPSASDWQTKVNQTISNANDLISRYGKSIMISEIGMDYNQPSAAKSFISDIKTKVRNLSGGKGLGVFYWEPEATPGYNGGYNKGAWQSDMKPTIALEGFLN

SEQ ID NO: 39 - protein, 316 aa, Cohnella laeviribosi
  REGION 1..316: note = mat_peptide
APAFAKGADISWVPGMEAQGYKWKDKNGVQRDIIDILKQDYQINSVRIRVFVNPSSDYGNGYLNKERAADLAQRAKNAGMSVMLTLHYSDSWADPGKQTKPAAWQNYTFEQLMDAVWNWTRDVMTTMQSRGVTPDWVQIGNETNNGMLWDDGKASVNMRNYAWLVNTGNNAVKSISSSTKTIVHLSNGYDNSLFVWNIGGLISNGATFDIIGMSLYPSASDWQTKVNQTISNANDLISRYGKSIMISEIGMDYNQPSAAKSFISDIKTKVRNLSGGKGLGVFYWEPEATPGYNGGYNKGAWQSDMKPTIALEGFLN

SEQ ID NO: 40 - protein, 324 aa, synthetic construct
  REGION 1..324: note = Mature sequence with His-tag
  REGION 1..324: note = mat_peptide
HHHHHHPRAPAFAKGADISWVPGMEAQGYKWKDKNGVQRDIIDILKQDYQINSVRIRVFVNPSSDYGNGYLNKERAADLAQRAKNAGMSVMLTLHYSDSWADPGKQTKPAAWQNYTFEQLMDAVWNWTRDVMTTMQSRGVTPDWVQIGNETNNGMLWDDGKASVNMRNYAWLVNTGNNAVKSISSSTKTIVHLSNGYDNSLFVWNIGGLISNGATFDIIGMSLYPSASDWQTKVNQTISNANDLISRYGKSIMISEIGMDYNQPSAAKSFISDIKTKVRNLSGGKGLGVFYWEPEATPGYNGGYNKGAWQSDMKPTIALEGFLN

SEQ ID NO: 41 - DNA, 3352 bp, Hamigera paravellanea
  sig_peptide 1..69
  mat_peptide 70..3349
  source 1..3352: mol_type = genomic DNA
  CDS 1..801
  CDS 873..1869
  CDS 1930..2223
  CDS 2297..2368
  CDS 2427..2514
  CDS 2578..3349
atgacgcgccttagtgagtgggctttcgtcctactctcaactttgggcgtcttcgcggctgctcaggcccaaacagtgtcgcaatggcccatccacgacaatgacttgaacacagtcgtccagtgggaccactacagcttcatcattaacggacagcgtatcttcgttttctcgggcgaattccactactggcgcattccggtccccgggttatggagggatatcctcgagaaggtcaaagcggccggattcactgcgtttgcattctactccagctgggcgtaccacgctccgaataaccacaccgtcgacttctcgacaggtgcccgtgatatcacgccgatctttgacctggccaaggagcttggtttgtacgtcatcgtccgtccggggccctacgtcaacgcggaagccaatgctggtggctaccctctttggctcaccaccggtgcttatggaagcctgaggaacaatgacacgcggtacatcaatgccttggaaccttacttttccaaggtgtcgcagatcacaagccagtatcagatcaccaacgaccacaacaccatctgctatcaaatcgagaacgagtatggccagcaatggatcggcagtgcatacgacagggttccgaatgagacggccattgcatacatggaaatcctcaaggcgagcgctcgcagaaatggcattgatattcctctcacggcgaatgacccgaacatgaacactcgttcgtgggggaaagactggtccgacgaaggtggaaacgtggacatccccggcgtcgactcctatccttcggtatgtggagactatgatcattttggaggtgaaccttttctgatgtttttttcttcatctccgtcttccagtgctggtcatgcgacctcagtgtatgcacttcgacaaacggagtatacgtcccgttccaggtcctgaactactacgactatttcgcagaaacgtcaccgacgatgccgtcattcatgccagaatttcagggtggctcttacaatccctggggcggtcccgaaggtggctgtccggacgacataggaccggaatttgcgaacctgttctacaggtggaacatcggtcagcgtgtcacggctatgagtttgtatatgctctatggaggaacaaactggggtgcaatggctgctcccgtgacagctagcagctatgactattctgctcccatctcagaggatcgctccatcggcgcgaaatactatgagaccaagctcctggggctgttcagtcggagcgcgcgagacctgaccgtgacggatctgatcggcaatggaacccagtataccaacaacgtgatgattcaggcacgcgaactcagaaacccggaaaccaatgccgctttctacgtcacagttcataccaacacctctgtttctactaacgaggtcttccacctgagagtcaacacctctgccggagctctaacgattcctaaacacgcgcttggcattcgactgaatggtcaccagtcgaagatcatagtgacggactttaccttcggccccaggactctgctctactcgaccgcagaagtcctcgcctatgccgcgctggacgacaccccaactctggctctctgggttccacctggagagtccggagagtttaacgtcaagggcgcaaaatcgggatcggtcaagaaatgccaggggtgttcgaacgtccagttccaccaggaaaacggtggtcttacagtcgccttcactcaatctcaagggatgagcgttgtggaactgaacgatggtagtcgcgtggttctgcttgacagggaatccgcataccgtttctgggctccagcattgactaacgatccattcgtgccggaggatgagactggtgcgtgttttccttatgccaatcgtgaaaaaaaaaaatgcttgctgacctgccaagcagttctgatccaaggcccctacctcgtccgcggggctaaactgtcaggctctacgctgtcggtaacaggtgatatcgtgaatgcaacgaccgtggagatcttcgcgcccaaaaccgtcaagtccattacctggaacgggagagaactgaagacttcgaagacgtcttatggcagtctgcagggctctttgaaggctcctgcacccgtcaaattgcccgctcttaccggctggaaatccaaggacagcttgcccgagcggcttgcatcatatgacgactctggtgcggcctgggttggtgagtagaagaaaatcataagcagttgaacggagcggaatagaacagaatcggtaaactgacatccaccaagatgccaaccacatgacaacattgaacccgagccctccagcaacacttccagtcctatacgccgacgaatatggtattgccgcctcctttccacctgtttccgacgatccgtcatactgactttcgtataggcttccacaacggcgtccgtctctggcgaggctacttcaacggcaccgctacgggggtcttcttgaacatccaaggaggaagcgccttgtaagctattcacaatcgccactcagcaaagcccgggtccaatactaacatctcgacacacagcggctggtcagcctacctcaacggccacttcctgggatcccatctcggcgccgcctccatcgcccaagccaaccgtaccctctccttcgccaacgccaccctcaatgcctttggccccaatgtcctcctcgtcatccacgacgacacaggccacgatcaaaccaccggtgccctgaacccgcgcggcattctgaacgcgaccctcctctccggcgacgactcggcccaattcactcactggcgcctcgccggcaccgccggcggcgaatccaacctcgaccccgtccgcggcgtgtacaacgaagacggcctcttcgccgagcgcgtcggctggcacctccccgggttcgacgactcggcttggcccgacgcctcgtctccgcgcgagggcttcgcgggcgcgaccgtccggttctaccggaccaccgtggccttagacctgccgcgggacgtggacgcgtcgatatcgttcgtgttctcgactcctccgtcgtcgtccgccgcgtaccgggcccagttgttcgtgaacggataccagtacggtcggtatcatccgcacatcggcaaccaggtcgtgtacccggttccaccgggcatcttggattaccagggcgacaacaccatcggggtcgcagtgtgggcgcagacggaggaaggggcacgggtggggttggactggcgcgtgaactatgtggcggatagttccttggatgtttctttcgacggggctgcgttgagaccggggtgggacgaggggcggttgcagtatgcatag

SEQ ID NO: 42 - protein, 1008 aa, Hamigera paravellanea
MTRLSEWAFVLLSTLGVFAAAQAQTVSQWPIHDNDLNTVVQWDHYSFIINGQRIFVFSGEFHYWRIPVPGLWRDILEKVKAAGFTAFAFYSSWAYHAPNNHTVDFSTGARDITPIFDLAKELGLYVIVRPGPYVNAEANAGGYPLWLTTGAYGSLRNNDTRYINALEPYFSKVSQITSQYQITNDHNTICYQIENEYGQQWIGSAYDRVPNETAIAYMEILKASARRNGIDIPLTANDPNMNTRSWGKDWSDEGGNVDIPGVDSYPSCWSCDLSVCTSTNGVYVPFQVLNYYDYFAETSPTMPSFMPEFQGGSYNPWGGPEGGCPDDIGPEFANLFYRWNIGQRVTAMSLYMLYGGTNWGAMAAPVTASSYDYSAPISEDRSIGAKYYETKLLGLFSRSARDLTVTDLIGNGTQYTNNVMIQARELRNPETNAAFYVTVHTNTSVSTNEVFHLRVNTSAGALTIPKHALGIRLNGHQSKIIVTDFTFGPRTLLYSTAEVLAYAALDDTPTLALWVPPGESGEFNVKGAKSGSVKKCQGCSNVQFHQENGGLTVAFTQSQGMSVVELNDGSRVVLLDRESAYRFWAPALTNDPFVPEDETVLIQGPYLVRGAKLSGSTLSVTGDIVNATTVEIFAPKTVKSITWNGRELKTSKTSYGSLQGSLKAPAPVKLPALTGWKSKDSLPERLASYDDSGAAWVDANHMTTLNPSPPATLPVLYADEYGFHNGVRLWRGYFNGTATGVFLNIQGGSAFGWSAYLNGHFLGSHLGAASIAQANRTLSFANATLNAFGPNVLLVIHDDTGHDQTTGALNPRGILNATLLSGDDSAQFTHWRLAGTAGGESNLDPVRGVYNEDGLFAERVGWHLPGFDDSAWPDASSPREGFAGATVRFYRTTVALDLPRDVDASISFVFSTPPSSSAAYRAQLFVNGYQYGRYHPHIGNQVVYPVPPGILDYQGDNTIGVAVWAQTEEGARVGLDWRVNYVADSSLDVSFDGAALRPGWDEGRLQYA

SEQ ID NO: 43 - protein, 985 aa, Hamigera paravellanea
  REGION 1..985: note = mat_peptide
QTVSQWPIHDNDLNTVVQWDHYSFIINGQRIFVFSGEFHYWRIPVPGLWRDILEKVKAAGFTAFAFYSSWAYHAPNNHTVDFSTGARDITPIFDLAKELGLYVIVRPGPYVNAEANAGGYPLWLTTGAYGSLRNNDTRYINALEPYFSKVSQITSQYQITNDHNTICYQIENEYGQQWIGSAYDRVPNETAIAYMEILKASARRNGIDIPLTANDPNMNTRSWGKDWSDEGGNVDIPGVDSYPSCWSCDLSVCTSTNGVYVPFQVLNYYDYFAETSPTMPSFMPEFQGGSYNPWGGPEGGCPDDIGPEFANLFYRWNIGQRVTAMSLYMLYGGTNWGAMAAPVTASSYDYSAPISEDRSIGAKYYETKLLGLFSRSARDLTVTDLIGNGTQYTNNVMIQARELRNPETNAAFYVTVHTNTSVSTNEVFHLRVNTSAGALTIPKHALGIRLNGHQSKIIVTDFTFGPRTLLYSTAEVLAYAALDDTPTLALWVPPGESGEFNVKGAKSGSVKKCQGCSNVQFHQENGGLTVAFTQSQGMSVVELNDGSRVVLLDRESAYRFWAPALTNDPFVPEDETVLIQGPYLVRGAKLSGSTLSVTGDIVNATTVEIFAPKTVKSITWNGRELKTSKTSYGSLQGSLKAPAPVKLPALTGWKSKDSLPERLASYDDSGAAWVDANHMTTLNPSPPATLPVLYADEYGFHNGVRLWRGYFNGTATGVFLNIQGGSAFGWSAYLNGHFLGSHLGAASIAQANRTLSFANATLNAFGPNVLLVIHDDTGHDQTTGALNPRGILNATLLSGDDSAQFTHWRLAGTAGGESNLDPVRGVYNEDGLFAERVGWHLPGFDDSAWPDASSPREGFAGATVRFYRTTVALDLPRDVDASISFVFSTPPSSSAAYRAQLFVNGYQYGRYHPHIGNQVVYPVPPGILDYQGDNTIGVAVWAQTEEGARVGLDWRVNYVADSSLDVSFDGAALRPGWDEGRLQYA

SEQ ID NO: 44 - DNA, 3391 bp, Aspergillus unguis
  sig_peptide 1..60
  mat_peptide 61..3388
  source 1..3391: mol_type = genomic DNA
  CDS 1..801
  CDS 847..1831
  CDS 1883..2176
  CDS 2236..2307
  CDS 2368..2458
  CDS 2527..3388
atggcgcgagtctttcaactgcttctcttcctcctgggaagctttcagcttctgacagcagctcagaacagctcccaaaccgaatggcctgtacatgacaacgggctaagcgaggtcgtccaatgggaccattacagcttttacgttcacggccagcggttcttcctgttctcaggggaatttcactactggcgaatcccagtcccggccttgtggcgcgacattttggagaaggtcaaggcgcttgggttcaccggctttgcgttctactcaagctgggcataccatgcgcccaacaaccacacggtcgacttctcgaccggtgcgcgcaacatcaagcacatctttgaccttgcagaggagcttggaatgtacattattgtgcgacccggaccgtacgtcaacgctgaagcctctgctggtgggtttccgctctggcttacaacaggcgcgtatgggtcgacaaggaacgacgatcctagatataccgcggcgtggaagccatatttttctaaggtgtctgagatcacgagcaggtatcaggtcacggatggtcacaatacgttgatttaccagatcgagaatgagtatgggcagcagtggatcggggatccggtcgatagggaccttaacgagacagctgctgcttatatggatttgttgaaagcgacagctcgtgaaaacggaatcaaggtgcccttgactgcgaacgatcctaacatgggatcaaaatcttggggcaacgactggtcggatgctgcagggaacgtcgatgctgtggggttggactcttatccttctgtgagtgctcagtctccataatcaagtcctgtctaatcgatcaagtgctggagctgcgacgtcagcgtctgcacaggaacgaacggagaatacgtaccataccaagtaataaactactacgactacttcaacgaagtccagccaagcatgcctttcttcatgcccgaattccaaggaggatcgtataatccatggggtggccctgagggtggctgtcccgaggacaccggagcggactttgccaacttgttctacaggtggaatatcgggcagcgcgagacagccataagtctgtacatgattttcgggggaacaaactggggtggtatcgccgcgccagtcaccgcaaccagttatgactactccgctcctatctcagaggatcgatcgataggctcaaagttctacgagacaaagctgctagccctgttcacacgagctgcgaaagatttgactgtgactgatcgtgtcggcaacggaacgcagtatacgagcaataaagccgtcagcgcaattgagctgcgcaaccctgagaccaatacgggtttttacgtgaccagccacttggacactacaaccggcacagacgaggccttcaagctgcacgtcaacacctccgaaggggcattcaccatcccaaggctaaatggcaccataaggcttaatggccatcaatcaaagattatcgtcaccgacttcaaattcggcttcaagacgcttttatactcaaccgcagaggttctcacctacgcagtctttgaccataaaccaactctcgtcctttgggttcccactggtgaatcaggcgaattcgcaatcaaaggcgcgaaatcaggttctgcttcgactgcgtcggtgcagttccatcggcacggaagaacactgactgttgggtttacccaggctaaaggcctgagtgttctggagcttgataatggcgtcagagtagttttgctggatagggaggcggcgtatacgttctgggcacctgccttgacggacaatccgcttgttcctgagggtgaaagtggtgagttcccttttttctctctcttaataatcggtgatgctaataaagtagtccttgtcagcggaccctacctcgtccgatcctccaaactatccggatcaaccctagctctacgaggtgactcgctgggcgaaacaacactagaagtctttgctccaaacaatgtaaagaaggtgacatggaacggaaagaaggtcaaggtgtctaggaccaaatacgggagcctgaaagccaacctcgccgaaccgcgctctgtggaactgcccgctctcgacggatggaaggtcagcgacagcctgccagagaggttctcagactatgatgactcgggcaaggcttgggttggtatgttacatactccgtatacctggatctttgaagagataaaatactgacatgagcagccgcaaaccatctgacaacacccaatcccaataaaccagcgactctccccgttctctacgccaatgaatatggtattccgcctgaactctaactcggatcaaccagatcatgagctaacaacttgattccaggcttccacaacggcgtccgcctctggcgcggctactttaactcctctactgcgacgggcgtcttcctaaacatccaaggcggcgctgcattgtacgtccaaccaaacccctgccttctgtaaagccagtcatgaacagacataatactaataaacccagcggttggtccgcctggcttaacggccagctcattggctcgcacctaggcaacgcgacgatcgaacaagccaacgcaacactcccattcccggacaacaccctctccaagaacggagaacagaatgtgctcctcgtcgtccacgatgacacgggacatgaccagacaacgggtgtgctcaacccacgaggaatcctcgaagcgcgtctcctctcagacagtgaagaagagaatgaagacgagcaaggaggattcacgcattggcgcgtcgcgggagctgcaggcggcgaatcgaacctcgatcccgtccgaggtgtgtataacgaggatggactctacgcggagcgtgtgggttggcatttacctgggttcgacgacagcgagtggtctctcgcagacaatgcgaaggcaccactagccttcaccggcgcaacagtcaagttcttccggactgtcatacccccgttatcgatcccagagggcctcgacgtctccatctcgtttgtgttttccacggcgaatgtgtcgtccatctcgaccaccaccaccacaaactcaacggttggagaagaaaacaaaggcgataaatcggccttccgcgctcaactcttcgtcaacggctaccagtacggacggtacaatccaattgtcgggaaccaagttgcgtatcctgtcccgccggggattttggactacaatgacgagaatacggttggggttgcagtttgggcacagacggaggccggagcggaattcgggctcgattggaaagtcgattatgtgcttgagagttcgctggatgttgtgaatttggatgtggaggggttgaggccgaggtggagtgaggagagggagagatttgcgtag

SEQ ID NO: 45 - protein, 1035 aa, Aspergillus unguis
MARVFQLLLFLLGSFQLLTAAQNSSQTEWPVHDNGLSEVVQWDHYSFYVHGQRFFLFSGEFHYWRIPVPALWRDILEKVKALGFTGFAFYSSWAYHAPNNHTVDFSTGARNIKHIFDLAEELGMYIIVRPGPYVNAEASAGGFPLWLTTGAYGSTRNDDPRYTAAWKPYFSKVSEITSRYQVTDGHNTLIYQIENEYGQQWIGDPVDRDLNETAAAYMDLLKATARENGIKVPLTANDPNMGSKSWGNDWSDAAGNVDAVGLDSYPSCWSCDVSVCTGTNGEYVPYQVINYYDYFNEVQPSMPFFMPEFQGGSYNPWGGPEGGCPEDTGADFANLFYRWNIGQRETAISLYMIFGGTNWGGIAAPVTATSYDYSAPISEDRSIGSKFYETKLLALFTRAAKDLTVTDRVGNGTQYTSNKAVSAIELRNPETNTGFYVTSHLDTTTGTDEAFKLHVNTSEGAFTIPRLNGTIRLNGHQSKIIVTDFKFGFKTLLYSTAEVLTYAVFDHKPTLVLWVPTGESGEFAIKGAKSGSASTASVQFHRHGRTLTVGFTQAKGLSVLELDNGVRVVLLDREAAYTFWAPALTDNPLVPEGESVLVSGPYLVRSSKLSGSTLALRGDSLGETTLEVFAPNNVKKVTWNGKKVKVSRTKYGSLKANLAEPRSVELPALDGWKVSDSLPERFSDYDDSGKAWVAANHLTTPNPNKPATLPVLYANEYGFHNGVRLWRGYFNSSTATGVFLNIQGGAAFGWSAWLNGQLIGSHLGNATIEQANATLPFPDNTLSKNGEQNVLLVVHDDTGHDQTTGVLNPRGILEARLLSDSEEENEDEQGGFTHWRVAGAAGGESNLDPVRGVYNEDGLYAERVGWHLPGFDDSEWSLADNAKAPLAFTGATVKFFRTVIPPLSIPEGLDVSISFVFSTANVSSISTTTTTNSTVGEENKGDKSAFRAQLFVNGYQYGRYNPIVGNQVAYPVPPGILDYNDENTVGVAVWAQTEAGAEFGLDWKVDYVLESSLDVVNLDVEGLRPRWSEERERFA

SEQ ID NO: 46 - protein, 1015 aa, Aspergillus unguis
  REGION 1..1015: note = mat_peptide
AQNSSQTEWPVHDNGLSEVVQWDHYSFYVHGQRFFLFSGEFHYWRIPVPALWRDILEKVKALGFTGFAFYSSWAYHAPNNHTVDFSTGARNIKHIFDLAEELGMYIIVRPGPYVNAEASAGGFPLWLTTGAYGSTRNDDPRYTAAWKPYFSKVSEITSRYQVTDGHNTLIYQIENEYGQQWIGDPVDRDLNETAAAYMDLLKATARENGIKVPLTANDPNMGSKSWGNDWSDAAGNVDAVGLDSYPSCWSCDVSVCTGTNGEYVPYQVINYYDYFNEVQPSMPFFMPEFQGGSYNPWGGPEGGCPEDTGADFANLFYRWNIGQRETAISLYMIFGGTNWGGIAAPVTATSYDYSAPISEDRSIGSKFYETKLLALFTRAAKDLTVTDRVGNGTQYTSNKAVSAIELRNPETNTGFYVTSHLDTTTGTDEAFKLHVNTSEGAFTIPRLNGTIRLNGHQSKIIVTDFKFGFKTLLYSTAEVLTYAVFDHKPTLVLWVPTGESGEFAIKGAKSGSASTASVQFHRHGRTLTVGFTQAKGLSVLELDNGVRVVLLDREAAYTFWAPALTDNPLVPEGESVLVSGPYLVRSSKLSGSTLALRGDSLGETTLEVFAPNNVKKVTWNGKKVKVSRTKYGSLKANLAEPRSVELPALDGWKVSDSLPERFSDYDDSGKAWVAANHLTTPNPNKPATLPVLYANEYGFHNGVRLWRGYFNSSTATGVFLNIQGGAAFGWSAWLNGQLIGSHLGNATIEQANATLPFPDNTLSKNGEQNVLLVVHDDTGHDQTTGVLNPRGILEARLLSDSEEENEDEQGGFTHWRVAGAAGGESNLDPVRGVYNEDGLYAERVGWHLPGFDDSEWSLADNAKAPLAFTGATVKFFRTVIPPLSIPEGLDVSISFVFSTANVSSISTTTTTNSTVGEENKGDKSAFRAQLFVNGYQYGRYNPIVGNQVAYPVPPGILDYNDENTVGVAVWAQTEAGAEFGLDWKVDYVLESSLDVVNLDVEGLRPRWSEERERFA

SEQ ID NO: 47 - DNA, 3859 bp, Aspergillus tamarii
  sig_peptide 1..66
  mat_peptide 67..3856
  source 1..3859: mol_type = genomic DNA
  CDS 1..125
  CDS 189..243
  CDS 299..321
  CDS 371..415
  CDS 477..948
  CDS 1005..1139
  CDS 1191..1210
  CDS 1269..1289
  CDS 1342..1544
  CDS 1594..1686
  CDS 1743..1780
  CDS 1835..1985
  CDS 2051..2464
  CDS 2523..2816
  CDS 2886..3856
atgctcatctccaagaccgtgttcagcgggcttgccttgggggcgtcctttgttggcgtttctggtcagcagaattcaagccgttggccgttgcacgacaacggtttgacagacactgtagaatggtgggttcagtcaaattgcgaattcaaggctgtttggttggctctgacaccatggctatacagggatcactatagtttcttgattaatggtcagagacatttcgttttctctggagaggtttgtccgcccaatcccctatattctgtatattcaatacattaacatcatatagttccattactggcgtatccctgtgtaaggcaagagtcccacaacggcaacgctctagctaatggattaccagacccgaattatggagagatctactcgagaagatcaaagccgctgggtaggtagtctcagattcttgacgcccgttgtcaacaacacgctaataacgaattggatagtttcactgccttttccatctacaatcactggggatatcatacccccaagcccggcgttctcgacttcgagaacggggcccacaacttcacttcgatcatgactctagccaaagagataggtctctacatgattatccgaccgggcccatacgtcaatgcggaagccaatgctggcggtctccctctgtgggcaactacaggtgcctacggaaaactacgggataacgaccctcggtacttggaggctttgaccccatactgggctaacatttctaaaatcattgctcctcatctcatcaccaacggcggaaatgtcatcctgtatcagatcgagaatgagtacgccgagcagtggcttgacgaggaaacccaggagcccaacacgtctggtcaggaatacatgcagtatttggaggacgttgctcgggaaaacggcattgatgctcctctgatccataatcttccgaacatggtagggcaatacgctcgcttgctgaagatacagaatttttggctgatacatagcagaacggtcactcatggtccaaggacctctccaacgctactggaaatgtcgatgtcattggcgtggacagctatcccacttgctggacctgcaatgtcagtgagtgtctctcaactaacggagagtatatcccatatgtaagtaacgcctgcctttctttggtgatttattatactaaactctctcagaaaaccttgacctactacgagtaagtgcaatagtacacggatttgtatgagtgaaacactaatttaccctcaaatcagctacttcaagaaactatcaccgtaagctttgccctctctgagactatctacacattctaattctctattacagcactcagccaagctttatgcccgagttccaaggcggttcatacaacccatggggtggaccccaaggaggctgcccggatgatcttggcccggatttcgcgaacctcttctaccgaaacctaatctatcagagagtcagtgctatctcgctgtacatgttatacggcggtacaaactggggctggcacggctcaacagatgtcggtgagttattcccaagtcgaatttatgccacaggtgctgatgagcccagcgacaagttacgattactcttctccaatttcggagaaccgaaagcttattgagaaatactacgagacaaaagtgctcactcaattcacgaaaagtacgcctcttttagtacgatatgtggaagcttgccaagctaacctcatgatacagtcgcccgggatctgtctaaagtcgatcgtttaggcaacgtaagtagagcagaacaatatcgtctacagagaaacgctaacaggggtcaacagagcacgagatattcaagtaacccagctgtttcagtttctgagctgcgaaatcctgacaatggcgcggctttctacgtaactcagcacgaatacactccatctggaacggtcgaaaagttcacagtcaaggttaacacatccgatggtgctcgtatgttacctcctgcggtctgaatttggtatatcacaatgataatctgctaattactcgacaagtcactattcctcaatacggctcccaaatcactctcaatggtcaccagtccaagattatcgtcacagacttcaacttcggctcgaagacgctcctttactctacggcagaagttcttacctatgctgttattgatggtaaagaagtgctggctctctgggtcccgactggtgaatctggagagttcaccgtgaagggagtgaattcggccaagttcgccgacaaaggacgcactgcgaacatcgagattcgccccggagcaaacaaggtgacagtatctttcatgcagagagcgggtatgagcgtggttgagcttggtgatggaacacgcattgttcttctcgatcggtctgctgctcatgtattctggtctcctccactcaacaatgaccctgccgaggccggcaacaacactggtaagtccacatcgatggcgttatacaaacagttgatagactcgctgacatgcttcagtcctcgtccatggtccctacttagttcgctcggctagattggaaggctgtgacttgaagctcactggagatatccagaattctacaaaggtcagcatctttgcgcccaattcggtatgctccgtcaattggaatggcaagaagacatccgtcaagtcagcgaagggtggtgtcataaccacaaccttgggaggcgatgccaagttcgaacttcccacgatctccggctggaagtatgcggacagtctccctgaaatcgcgaaggactattccgctacaagcaaggcttgggttggtatgttatttctctcctcctcggtcgccaatagcacccgccagtgccagctaacaacagaaaaaccagtggctacgaagacaaactcgtctaatccgactcccccggcaccaaacaacccagtcctctacgtggacgagaacgatatccacgtcggcaaccacatctaccgcgccactttccccagcaccgacgagcccccaaccgacgtctacctcaacatcaccggaggtcgcgcattcggctactctgtctggctgaactcagaattcatcggctcctggctcggcaccccgacaaccgagcagaacgaccagacattctcattctccaacgcaaccctcagcacagacggagacaacatcctagtcgtcgtcatggacaactcggcccacgatctgcgcgagggagcaaccgacccccgaggaatcacaaacgccactctcgtcggtcccggaacctactccttcaccgagtggaaactcgccggcaacgcaggcttcgaagaccaccttgatccggtccgcgccccgctcaacgagggcagtctgtacgccgagcgagtcggtatccatctcccgggatatcagttcgacgaggccgaagaggtgccttcgaacagcacgagcctaaccgttcccggtgctggtattcgcgtcttccgcaccgttgttcccctctccgtgccccagggactggacgtctctatctcgttccgtttgactgctccctcgaatgtgacctttacctctacggagggatacaccaaccagctgcgcgctctgctcttcgttaatggataccagtatggtcgctttaacccttacatcggtcatcagattgacttccctgttcctccgggcgtccttgattataatggggataacacgattgcggtgacggtgtggagtcagagtgtggatggtgctgagatgaaaattgattggaatgtggactatgtccatgagaccagcttcgacatgaactttgacggagcatacctgagacctggatggatcgaggagagacgtgaatatgcttaa

SEQ ID NO: 48 - protein, 1020 aa, Aspergillus tamarii
MLISKTVFSGLALGASFVGVSGQQNSSRWPLHDNGLTDTVEWDHYSFLINGQRHFVFSGEFHYWRIPVPELWRDLLEKIKAAGFTAFSIYNHWGYHTPKPGVLDFENGAHNFTSIMTLAKEIGLYMIIRPGPYVNAEANAGGLPLWATTGAYGKLRDNDPRYLEALTPYWANISKIIAPHLITNGGNVILYQIENEYAEQWLDEETQEPNTSGQEYMQYLEDVARENGIDAPLIHNLPNMNGHSWSKDLSNATGNVDVIGVDSYPTCWTCNVSECLSTNGEYIPYKTLTYYDYFKKLSPTQPSFMPEFQGGSYNPWGGPQGGCPDDLGPDFANLFYRNLIYQRVSAISLYMLYGGTNWGWHGSTDVATSYDYSSPISENRKLIEKYYETKVLTQFTKIARDLSKVDRLGNSTRYSSNPAVSVSELRNPDNGAAFYVTQHEYTPSGTVEKFTVKVNTSDGALTIPQYGSQITLNGHQSKIIVTDFNFGSKTLLYSTAEVLTYAVIDGKEVLALWVPTGESGEFTVKGVNSAKFADKGRTANIEIRPGANKVTVSFMQRAGMSVVELGDGTRIVLLDRSAAHVFWSPPLNNDPAEAGNNTVLVHGPYLVRSARLEGCDLKLTGDIQNSTKVSIFAPNSVCSVNWNGKKTSVKSAKGGVITTTLGGDAKFELPTISGWKYADSLPEIAKDYSATSKAWVVATKTNSSNPTPPAPNNPVLYVDENDIHVGNHIYRATFPSTDEPPTDVYLNITGGRAFGYSVWLNSEFIGSWLGTPTTEQNDQTFSFSNATLSTDGDNILVVVMDNSAHDLREGATDPRGITNATLVGPGTYSFTEWKLAGNAGFEDHLDPVRAPLNEGSLYAERVGIHLPGYQFDEAEEVPSNSTSLTVPGAGIRVFRTVVPLSVPQGLDVSISFRLTAPSNVTFTSTEGYTNQLRALLFVNGYQYGRFNPYIGHQIDFPVPPGVLDYNGDNTIAVTVWSQSVDGAEMKIDWNVDYVHETSFDMNFDGAYLRPGWIEERREYA

SEQ ID NO: 49 - protein, 998 aa, Aspergillus tamarii
  REGION 1..998: note = mat_peptide
QQNSSRWPLHDNGLTDTVEWDHYSFLINGQRHFVFSGEFHYWRIPVPELWRDLLEKIKAAGFTAFSIYNHWGYHTPKPGVLDFENGAHNFTSIMTLAKEIGLYMIIRPGPYVNAEANAGGLPLWATTGAYGKLRDNDPRYLEALTPYWANISKIIAPHLITNGGNVILYQIENEYAEQWLDEETQEPNTSGQEYMQYLEDVARENGIDAPLIHNLPNMNGHSWSKDLSNATGNVDVIGVDSYPTCWTCNVSECLSTNGEYIPYKTLTYYDYFKKLSPTQPSFMPEFQGGSYNPWGGPQGGCPDDLGPDFANLFYRNLIYQRVSAISLYMLYGGTNWGWHGSTDVATSYDYSSPISENRKLIEKYYETKVLTQFTKIARDLSKVDRLGNSTRYSSNPAVSVSELRNPDNGAAFYVTQHEYTPSGTVEKFTVKVNTSDGALTIPQYGSQITLNGHQSKIIVTDFNFGSKTLLYSTAEVLTYAVIDGKEVLALWVPTGESGEFTVKGVNSAKFADKGRTANIEIRPGANKVTVSFMQRAGMSVVELGDGTRIVLLDRSAAHVFWSPPLNNDPAEAGNNTVLVHGPYLVRSARLEGCDLKLTGDIQNSTKVSIFAPNSVCSVNWNGKKTSVKSAKGGVITTTLGGDAKFELPTISGWKYADSLPEIAKDYSATSKAWVVATKTNSSNPTPPAPNNPVLYVDENDIHVGNHIYRATFPSTDEPPTDVYLNITGGRAFGYSVWLNSEFIGSWLGTPTTEQNDQTFSFSNATLSTDGDNILVVVMDNSAHDLREGATDPRGITNATLVGPGTYSFTEWKLAGNAGFEDHLDPVRAPLNEGSLYAERVGIHLPGYQFDEAEEVPSNSTSLTVPGAGIRVFRTVVPLSVPQGLDVSISFRLTAPSNVTFTSTEGYTNQLRALLFVNGYQYGRFNPYIGHQIDFPVPPGVLDYNGDNTIAVTVWSQSVDGAEMKIDWNVDYVHETSFDMNFDGAYLRPGWIEERREYA

SEQ ID NO: 50 - DNA, 3197 bp, Curvularia spicifera
  sig_peptide 1..81
  mat_peptide 82..3194
  source 1..3197: mol_type = genomic DNA
  CDS 1..265
  CDS 320..917
  CDS 973..1925
  CDS 1981..3194
atgaagactttcgttgggctctcgtggctgtcggccttgtcttcgttggtgacgctcccaaatggctccggtgttgctgcccagaacaacacgcctagtacgtggccgctccacgacaatggtctgaatgatgtcgtacaatgggatcattattcctttaaagtgaacggaaagcgccttttcgttttctctggagaaattcactactggcgtatcccggtctatgaggtttgggaggacttgttagaaaaaattaaggcggctggtaagtatttccatttgcataagatgcatgtcgattacggctgacgaccattaggtttcacggctttcgccttctacggcaactgggcctatcacagcgcaaacaaccagaccttggactttgaaagcggcgcgcacgactttacgaagctcttcgagatcgcggagcgcgtcggcctttacgtcattaccaggcctggtccttatgtcaatgctgaggcgaacgctggaggcttcccattatggctcactacgggagcttatggaacgctacgcaacgacgaccccagatacctccaagcattggacccttacttctccaagttctctgagctcacatccaagcatctcgtgaccaagggcggaaaagcgcttgtctaccagatcgagaacgagtatggtgagcagtggaagaatagagaccagaagattcccaatgaaagtgccggaagatatatgcaggcgcttgaggatttggcacgggctcatggcattgacgtccccctaatccacaacgaccccaatatgaacaccaagagctggagcaaagactatgcccctggtgctgtaggaaatgtcgatgttgctgggctcgacagctacccatcctgttggtcctgcaacctggatgagtgcacgggtaccaatggagagtaagtgttgtaaatctcaaacgctccagtaacagttactaacgttatgttctagatacgtagcataccaaaccatcaactactttgatcatttcgaagaagtatctccaacccagccaagcttcttccctgaattccaaggtggttcgtacaatccttggggtggacccgaaggtggctgtcccggtgacattggagctgatttcgcaaatctcttctaccgaaacctggtctcccaacgcgttaccgcaatctcactttatatggtttttggcggcacaaattggggcgccattgcagccccagtcacagccacgtcgtatgactatagcagtcctatcagcgagaaccgggagattggcgccaaattctacgagacgaagaacttggctttgttcactcgtgttgcggaagacttgacagttaccgatcgccttggaaattctacttcttacacgaccaactcggcagtcgaggcgagtgaactccgcaacccacacaccaacggcgcattttacgttaccattcatgccacatcgtcttccgcgacgaaggaatcattcaagctccatgtgagcacatccatcggtaatctcactatccctcaacatgctggttctattgttctcgatggccatcaatccaagatccttgttaccgatttcgcaatgggcaacagtaccttgacatactccactgcagaagttgtcacctacgctcttatcgactccaagccagttgttttgctatcaactggtattggcgagtctgctgaattccatgtcaagggcgctaagaagggttccgctgtcagcagtggtgctagctcgaatgctacgttctacaccgaggccggtggtgttacgaccagcatacagaaagtttcgggtatgagcgtctaccagttcgataatggtgtgaaggttgttgttgcggataagcctaccgcgtacctgttctgggcacctaacctgtcgaacgacccctttgcgcccgttgatcaatccggtaagtatactaaattcgtgattcttctggttctcgaaatctaacatgcacatagttttggtccagggaccatacctcgtccgccacgtagctctcgacggccacgtcctcgccctgaaaggagatatcatgaacagcactgacatcgaagtctttgcctgtcacaatgccaaaactctgtcctggaatggaaagaagctctctacctcgcgaacctcgtacggtagtctgaaagcccacatcaccgctttcaacggcactattcagctaccttccctcgacaactggaaagtcaacgaaggtctcccagagaaggaggcagattacgatgacagcagcgccgcttgggttatagccgaccacctcagcacccccaaccctaccaagcccgacactcttcccgttctgtacgtcgatgagtatggcttccacaacagcttccaccttttccgcggctacttcgatggctccgccaccggcgtccaactctctgtgcaaggcggtctcgcatttggctggagtgcctggctaaacggcaaacatattggttcttggctgggcaatacgaccctcggtgtaggcaacgcaacgctctcctttgccaacgccacagttcactccaatggaaccaacgtcctcctcgtcgcccaagacaacacaggccacgatctccgcggcggcgccaccgatccccgcggtatcctgcgcgcatccctttccggcccctcaaacttcacaagctggaaaatcgcaggtgaagccggcggcgaatccatccagctcgaccccgtccgtggtcccctggctgaaggcggcctcgtcgctgaacgccttggctggcacctccctggcttcgacgacgcggactgggccaccagctcgccttccgccggattctcaggcgcagatataaagttctaccgtactacattcccgcttgatgtacctgaccatgttgatgcttccttcgcatttgtgctgaacgcccctgctgcgaagacgattcgcgtccagctttttgtcaatgggtatcagtatgcgcggtttaatccgtatgtgggtaatgaaatcaagttccctgttcctccgggcattctcaactacagcggagagaatgtggttgggctgagtgtgtgggcacaagaggaagacggagcaaaggtcgatgtgcgtatggtgcaggagtttgcggttgaaagtagttggaaatcgaggtttaatggcgagtatttgaggccgaagtggacagaggagagactggagtatgcttga

SEQ ID NO: 51 - protein, 1010 aa, Curvularia spicifera
MKTFVGLSWLSALSSLVTLPNGSGVAAQNNTPSTWPLHDNGLNDVVQWDHYSFKVNGKRLFVFSGEIHYWRIPVYEVWEDLLEKIKAAGFTAFAFYGNWAYHSANNQTLDFESGAHDFTKLFEIAERVGLYVITRPGPYVNAEANAGGFPLWLTTGAYGTLRNDDPRYLQALDPYFSKFSELTSKHLVTKGGKALVYQIENEYGEQWKNRDQKIPNESAGRYMQALEDLARAHGIDVPLIHNDPNMNTKSWSKDYAPGAVGNVDVAGLDSYPSCWSCNLDECTGTNGEYVAYQTINYFDHFEEVSPTQPSFFPEFQGGSYNPWGGPEGGCPGDIGADFANLFYRNLVSQRVTAISLYMVFGGTNWGAIAAPVTATSYDYSSPISENREIGAKFYETKNLALFTRVAEDLTVTDRLGNSTSYTTNSAVEASELRNPHTNGAFYVTIHATSSSATKESFKLHVSTSIGNLTIPQHAGSIVLDGHQSKILVTDFAMGNSTLTYSTAEVVTYALIDSKPVVLLSTGIGESAEFHVKGAKKGSAVSSGASSNATFYTEAGGVTTSIQKVSGMSVYQFDNGVKVVVADKPTAYLFWAPNLSNDPFAPVDQSVLVQGPYLVRHVALDGHVLALKGDIMNSTDIEVFACHNAKTLSWNGKKLSTSRTSYGSLKAHITAFNGTIQLPSLDNWKVNEGLPEKEADYDDSSAAWVIADHLSTPNPTKPDTLPVLYVDEYGFHNSFHLFRGYFDGSATGVQLSVQGGLAFGWSAWLNGKHIGSWLGNTTLGVGNATLSFANATVHSNGTNVLLVAQDNTGHDLRGGATDPRGILRASLSGPSNFTSWKIAGEAGGESIQLDPVRGPLAEGGLVAERLGWHLPGFDDADWATSSPSAGFSGADIKFYRTTFPLDVPDHVDASFAFVLNAPAAKTIRVQLFVNGYQYARFNPYVGNEIKFPVPPGILNYSGENVVGLSVWAQEEDGAKVDVRMVQEFAVESSWKSRFNGEYLRPKWTEERLEYA

SEQ ID NO: 52 - protein, 983 aa, Curvularia spicifera
  REGION 1..983: note = mat_peptide
QNNTPSTWPLHDNGLNDVVQWDHYSFKVNGKRLFVFSGEIHYWRIPVYEVWEDLLEKIKAAGFTAFAFYGNWAYHSANNQTLDFESGAHDFTKLFEIAERVGLYVITRPGPYVNAEANAGGFPLWLTTGAYGTLRNDDPRYLQALDPYFSKFSELTSKHLVTKGGKALVYQIENEYGEQWKNRDQKIPNESAGRYMQALEDLARAHGIDVPLIHNDPNMNTKSWSKDYAPGAVGNVDVAGLDSYPSCWSCNLDECTGTNGEYVAYQTINYFDHFEEVSPTQPSFFPEFQGGSYNPWGGPEGGCPGDIGADFANLFYRNLVSQRVTAISLYMVFGGTNWGAIAAPVTATSYDYSSPISENREIGAKFYETKNLALFTRVAEDLTVTDRLGNSTSYTTNSAVEASELRNPHTNGAFYVTIHATSSSATKESFKLHVSTSIGNLTIPQHAGSIVLDGHQSKILVTDFAMGNSTLTYSTAEVVTYALIDSKPVVLLSTGIGESAEFHVKGAKKGSAVSSGASSNATFYTEAGGVTTSIQKVSGMSVYQFDNGVKVVVADKPTAYLFWAPNLSNDPFAPVDQSVLVQGPYLVRHVALDGHVLALKGDIMNSTDIEVFACHNAKTLSWNGKKLSTSRTSYGSLKAHITAFNGTIQLPSLDNWKVNEGLPEKEADYDDSSAAWVIADHLSTPNPTKPDTLPVLYVDEYGFHNSFHLFRGYFDGSATGVQLSVQGGLAFGWSAWLNGKHIGSWLGNTTLGVGNATLSFANATVHSNGTNVLLVAQDNTGHDLRGGATDPRGILRASLSGPSNFTSWKIAGEAGGESIQLDPVRGPLAEGGLVAERLGWHLPGFDDADWATSSPSAGFSGADIKFYRTTFPLDVPDHVDASFAFVLNAPAAKTIRVQLFVNGYQYARFNPYVGNEIKFPVPPGILNYSGENVVGLSVWAQEEDGAKVDVRMVQEFAVESSWKSRFNGEYLRPKWTEERLEYA

SEQ ID NO: 53 - DNA, 3829 bp, Aspergillus oryzae
  sig_peptide 1..66
  mat_peptide 67..3826
  source 1..3829: mol_type = genomic DNA
  CDS 1..125
  CDS 195..249
  CDS 306..328
  CDS 378..422
  CDS 481..952
  CDS 1009..1143
  CDS 1193..1212
  CDS 1266..1286
  CDS 1337..1539
  CDS 1588..1680
  CDS 1735..1772
  CDS 1826..1976
  CDS 2035..2448
  CDS 2507..2800
  CDS 2856..3826
atgctcatctccaagaccgtgctcagcggacttgccttgggggcgtccttcgttggcgtttctgctcagcagaactcaacccgttggccgttgcatgacaacggcttgacagacactgtagaatggtaggtttagccaatttgtggattcatttgtggatcaatactgttagctctgacaccatggctatacagggatcactatagtttcttgattaatggtcagagacattttgttttctctggagaggttggtccacccaatcgtttatgttctacatggttcaatgcattaacatcgtatagttccattactggcgtattcctgtgtaaggcaagagtcctacaacggcagcgctctcgctaatatataaccaggcccgaattatggagagatctactggagaagatcaaggccgctgggtaggtagttccagattttgaaagtcgtttctcggcacgctaatggcaaattcgacagtttcactgccttttccatctacaatcactggggataccacagccctaaacccggtgttctcgactttgagaacggagcccacaatttcacctcgatcatgactctagccaaagagataggtctctacatgatcatccggccgggcccatacgtcaatgcagaagccaatgctggcggtctccctctgtggacgactacaggtgcctacgggaaactgcgggataacgaccctcggtatctggaggctttgaccccgtactgggctaacatttctaaaattattgcccctcatctcatcactaatgacggaaatgtaatcctgtatcagatcgaaaatgagtacgccgagcagtggcttgatgaggaaacccacgagcccaacacgtctggtcaggaatacatgcagtatttggaggatgttgctcgggaaaatggcattgatgctcctctgatccataatcttcccaacatggtagggcaatatgctcacttactgaagatacagaatatttggctgatgtataacagaacggtcactcatggtccaaggacctctccaacgccaccggaaatgtcgatgtcattggcgtggacagctatcccacttgctggacctgcaatgtcagtgagtgtgcttcaactaacggagagtatatcccatatgtaagtaggactttgtctttgtctggaggttcatgctaatttacctcagaaaaccttgatctactacgagtaagtgtgatgcacagactgtacgagttaaaactgacttaccctcaaattagctactttaaggaattatcaccgtgagtttgctctacttgagactacccacacattctaacgcctatcatagcactcaaccaagcttcatgcccgagttccaaggcggctcgtacaacccatggggtggacctcaaggcggctgcccggatgaccttggcccggattttgcgaatctcttctaccgaaacttgatctcccagagagtcagcgctatctcgttgtacatgttgtacggcggtaccaactggggctggcacgcctcaacggatgtcggtaagttatccccaatccaacttatgctataggtgttgatgagcccagcgacgagctacgactactcctccccaatttcggagaaccgaaagctcattgagaaatactatgagacgaaagtactcactcaattcacgaaaagtacgcctctttatccgataggtggaagctcgccaagctaatctcaggatacagtcgcccaggatctgtctaaggtcgaccggttaggcaacgtaagtagatgataacaatatcgtgtaccgagaaacattaaccaagttaatagagcacgaaatactcgagcaatccagcagtgtcggttgctgagctgcggaaccctgacactggcgcggctttctacgtaactcagcacgagtacactccatctggaacggttgaaaagttcacggtcaaggttaacacttccgagggtgctcgtatgttatctcctctagtacccatatcgcaatgatcaactgctgacttcttgacaagttactattcctcagtatggctcccaaatcactctcaacggtcaccaatccaagatcattgtcacggacttcaagttcggctcgaagacactcctttactctacggcggaggttcttacctacgctgttattgatggcaaagaagtgctggctctctgggtccctactggagaatcgggagaattcaccgtgaagggagtgaattcggctaagttcgccgacaaagggcgtactgcgaacatcgagattcaccctgggacaaacaatgtaacagtctctttcatgcagagatcgggtatgagcctggttgagcttggtgatggaacacgcattgttcttctcgatcggtctgctgctcatgtattctggtctactccactcaacaatgaccctgccgaggctggcaacaacactggtgagtccccatcgatggcggtatacaaacagttgataggctcgctgacactcctcagtccttgtccatggcccctacttagttcgctcggctaaactggaaggctgtgacttgaaactcactggagatatccagaactctacagaggtcagcatctttgcacccaagtctgtatgctctgtcaattggaatggcaagaagacatccgtcaagtcggcgaagggtggtgttataaccacaaccctgggaggcgatgccaagttcgagcttcccacgatctctggctggaagtctgcggacagtctccctgaaatcgcaaaggactactccgctacaagcaaggcttgggttggtatgttaccctctcctccacggccaatagtacccaccagctaacaaaagaccagtggctacaaagacaaactcgtctaaccctactcccccggcaccgaacaacccagtcctctacgtagacgagaacgatatccacgtcggcaaccacatctaccgcgccacattccccagcaccgacgagcctccaaccgacgtctacctcaacatcaccggaggtcgcgcattcggctactcagtctggctgaactccgacttcatcggctcctggctcggcactgcgacaactgagcaaaacgaccagacattctccttctccaacgcaaccctcagcacagacgaagacaacatcctagtcgtcgtcatggacaactcagcccacgacttgcgcgacggagcactcaacccccgaggcatcacaaacgccaccctcatcggtcccggaagctactccttcaccgagtggaaactggccggcaacgcaggcttcgaagaccaccttgacccggtccgcgccccgctcaacgagggcagtctgtacgccgagcgcgtcggtatccatctcccgggctatgagttcgacgaagccgaggaggtgtcttcaaacagcacgagcctaaccgttcccggcgctggtattcgcgtcttccgcactgttgttcccctctccgtgccccagggactggacgtctctatctcgttccgtctgacggcgccctcgaacgtaacctttacctctgcggaggggtatactaaccagctgcgggctctgcttttcgtcaatgggtaccagtatggtcgctttaacccctatatcggtcatcagatcgacttccctgttcctccgggtgtccttgattacaacggggataacacgattgccgtgacggtgtggagtcagagtgtggatggtgctgagatcaaggtcgattggaatgtggactatgtccatgagaccagcttcgatatgaactttgatggagcgtacctgagacctggatggatcgaggagagacgtgaatatgcttaa

SEQ ID NO: 54 - protein, 1020 aa, Aspergillus oryzae
MLISKTVLSGLALGASFVGVSAQQNSTRWPLHDNGLTDTVEWDHYSFLINGQRHFVFSGEFHYWRIPVPELWRDLLEKIKAAGFTAFSIYNHWGYHSPKPGVLDFENGAHNFTSIMTLAKEIGLYMIIRPGPYVNAEANAGGLPLWTTTGAYGKLRDNDPRYLEALTPYWANISKIIAPHLITNDGNVILYQIENEYAEQWLDEETHEPNTSGQEYMQYLEDVARENGIDAPLIHNLPNMNGHSWSKDLSNATGNVDVIGVDSYPTCWTCNVSECASTNGEYIPYKTLIYYDYFKELSPTQPSFMPEFQGGSYNPWGGPQGGCPDDLGPDFANLFYRNLISQRVSAISLYMLYGGTNWGWHASTDVATSYDYSSPISENRKLIEKYYETKVLTQFTKIAQDLSKVDRLGNSTKYSSNPAVSVAELRNPDTGAAFYVTQHEYTPSGTVEKFTVKVNTSEGALTIPQYGSQITLNGHQSKIIVTDFKFGSKTLLYSTAEVLTYAVIDGKEVLALWVPTGESGEFTVKGVNSAKFADKGRTANIEIHPGTNNVTVSFMQRSGMSLVELGDGTRIVLLDRSAAHVFWSTPLNNDPAEAGNNTVLVHGPYLVRSAKLEGCDLKLTGDIQNSTEVSIFAPKSVCSVNWNGKKTSVKSAKGGVITTTLGGDAKFELPTISGWKSADSLPEIAKDYSATSKAWVVATKTNSSNPTPPAPNNPVLYVDENDIHVGNHIYRATFPSTDEPPTDVYLNITGGRAFGYSVWLNSDFIGSWLGTATTEQNDQTFSFSNATLSTDEDNILVVVMDNSAHDLRDGALNPRGITNATLIGPGSYSFTEWKLAGNAGFEDHLDPVRAPLNEGSLYAERVGIHLPGYEFDEAEEVSSNSTSLTVPGAGIRVFRTVVPLSVPQGLDVSISFRLTAPSNVTFTSAEGYTNQLRALLFVNGYQYGRFNPYIGHQIDFPVPPGVLDYNGDNTIAVTVWSQSVDGAEIKVDWNVDYVHETSFDMNFDGAYLRPGWIEERREYA

SEQ ID NO: 55 - protein, 998 aa, Aspergillus oryzae
  REGION 1..998: note = mat_peptide
QQNSTRWPLHDNGLTDTVEWDHYSFLINGQRHFVFSGEFHYWRIPVPELWRDLLEKIKAAGFTAFSIYNHWGYHSPKPGVLDFENGAHNFTSIMTLAKEIGLYMIIRPGPYVNAEANAGGLPLWTTTGAYGKLRDNDPRYLEALTPYWANISKIIAPHLITNDGNVILYQIENEYAEQWLDEETHEPNTSGQEYMQYLEDVARENGIDAPLIHNLPNMNGHSWSKDLSNATGNVDVIGVDSYPTCWTCNVSECASTNGEYIPYKTLIYYDYFKELSPTQPSFMPEFQGGSYNPWGGPQGGCPDDLGPDFANLFYRNLISQRVSAISLYMLYGGTNWGWHASTDVATSYDYSSPISENRKLIEKYYETKVLTQFTKIAQDLSKVDRLGNSTKYSSNPAVSVAELRNPDTGAAFYVTQHEYTPSGTVEKFTVKVNTSEGALTIPQYGSQITLNGHQSKIIVTDFKFGSKTLLYSTAEVLTYAVIDGKEVLALWVPTGESGEFTVKGVNSAKFADKGRTANIEIHPGTNNVTVSFMQRSGMSLVELGDGTRIVLLDRSAAHVFWSTPLNNDPAEAGNNTVLVHGPYLVRSAKLEGCDLKLTGDIQNSTEVSIFAPKSVCSVNWNGKKTSVKSAKGGVITTTLGGDAKFELPTISGWKSADSLPEIAKDYSATSKAWVVATKTNSSNPTPPAPNNPVLYVDENDIHVGNHIYRATFPSTDEPPTDVYLNITGGRAFGYSVWLNSDFIGSWLGTATTEQNDQTFSFSNATLSTDEDNILVVVMDNSAHDLRDGALNPRGITNATLIGPGSYSFTEWKLAGNAGFEDHLDPVRAPLNEGSLYAERVGIHLPGYEFDEAEEVSSNSTSLTVPGAGIRVFRTVVPLSVPQGLDVSISFRLTAPSNVTFTSAEGYTNQLRALLFVNGYQYGRFNPYIGHQIDFPVPPGVLDYNGDNTIAVTVWSQSVDGAEIKVDWNVDYVHETSFDMNFDGAYLRPGWIEERREYA

SEQ ID NO: 56 - DNA, 3355 bp, Aspergillus carneus
  sig_peptide 1..60
  mat_peptide 61..3352
  source 1..3355: mol_type = genomic DNA
  CDS 1..801
  CDS 870..1866
  CDS 1916..2215
  CDS 2267..2338
  CDS 2389..2476
  CDS 2530..3352
atggcgcgtctcccacagctcctcttcctactcctcgcgagtgtcgggctcctcagcgcagcccagaaccacaccgactccgaatggccactccacgataacggcctaaacaccgtcgttcaatgggatcactacagcttccaggtccacggccagcgcatcttcgtcttctccggcgaatttcactactggcgcatccccgtcccgggactctggcgcgacatcctggagaagatcaaggctgccggattcactgcattcgctttctactccagctgggcctaccatgcacccaacaatcacactgtggacttctcgaccggcgcccgcgacatcacccccatctacgagctcgcgaaagagctgggcatgtatatcatcgtccgaccgggcccctacgtcaatgcggaggccagcgccggcggctatcccctgtgggtgaccaccggtgcatacggcagtctgcggaacgacgacgcacggtacaccgaggcctggaagccgtactttgccaaaatgtcggaaatcacgagccagtaccaggtcaccgatggccacaatacgttctgctatcagattgagaacgagtacggccagcaatggattggagatcccgtcgatcgaaaccccaaccagacggccgttgcgtacatggaactcctcgaagagagtgcccgcgaaaatggcatcgtcgtgccattgactgcgaatgaccccaacatgaacaccaagtcctgggggaatgattggtctaatgcagggggcaatgtcgatgttgtcgggctggattcttacccttctgtaagctattctccctcctatacaacacccctatacaagatctcctgaccaacaaactaatgatacagtgctggacttgcgacgtcacccaatgcacctccaccaacggagaatacgtgccctacaaggtgatggggtactacgactacttccaggaggtgcagcccaccatgccgggcttcatgcctgagttccagggtgggagttacaacccctgggccggcccggagggtggatgtcccggagacacgggagtcgactttgcgaatctcttctaccggtggaacatcgcgcagcgggtgacggctatgagtctgtacatgctgtacgggggcacgaactggggcgccatcgccgcgccggtcacggctaccagctacgactactcctcgcccatctcggaagaccgctccatcggcagcaaatactacgagaccaagctcctggcgctcttcacccgcagtgccacggacctgaccatgaccgaccgcatcggaaacggcacgcagtacacgaacaacccggctgtcgccgcctacgaactgcgtaaccccgtcaccaacggggcgttttacgtgaccatccatgcagacagcaccgtcggctcggatgagtcgttccggttgaacgtcaacacctccgcaggtgcgttcacggtccccagcaagggcgcaatccgtctcaacggacaccaatcgaagattgtcgtcacggacttccgcttcgggccctctcactcgttgctgtattccaccgcggaggtcctcacccatgcggtgttcgacaagcaggccactatcgtcctttgggttcccaccggggagtcgggcgaattcgccgtcaagggcgcaaagtccggtaaggtagaaagctgtccacggtgctccaacgcgaccttcactcggaagaaagatgtgctcgttgtcaactttacgcagactggcgggatgagtgtgctccagctgaacaacggcgtgcgcgtcgttcttcttgatcgtcccgctgcatacaacttctgggctcctccggtgaccgacgatccttttgccccagagaccgatctgggtaagatggcttcgcccttctaaggtcacaattcgttaacagtaggcagttctcgtccaaggcccatacctcgtgcgttccgcgagtctgtccgggtcgaccctcgcgctgagaggcgactcgatcaaagagaccgcgttggagatcttcgcacccaagaaggtgaagacagtcacctggaatgggaagcgagtcaagacttccaagtcatcatacgggagtctcaccgcgtcgctcgcacctccaccggctgtgacgctcccggcattgacctcgacccgatggaagtcccaagacagtctgcccgaaaggcttccatcctacgacgactccggaccggcctgggttggtacgtatctcgctacattctctctatgtcccgtactaacaacctacgcagacgccgaccacatgactacacagaaccccaggaccccggagaccctccccgtgctctacgcagatgaatacggtactatcaccctcactcacattccctcaaacacctcactaacggtacaggcttccacaatggcatccgcctctggcgcgggtccttcaccgacgctgcctcgggcgtctacctcaacgtccaaggcggcgccgccttgtacgtacattccctcctcatccctcccagcaccaactaacatacattcccagtggctggtccgcctacctgaacggccacttcctcggctcccacctcggcacagcaacaacctcccaggcgaacaaaacgctcgtcttcccaaccggtgcactcaaccaaaacgccaccaacaccctcctcgtcatccatgacgacaccggccacgaccagaccaccggcgcgctgaacccgcgcggcatcctcgccgcccggctgctccccgcctccaacgccgcggccgactcgaccgccccgaccttcacacggtggcgcgtcgccggcacagcgggcggggaatccgacctcgaccccgtacgcggcgtctacaacgaagacgggctcttcgcggagcgcgtcggctggcacctccccggcttcgacgacggcgcctggcccgccgccaacacgaccgccgtggcgcaagaaaccggaaccgtgtcgctgtccttcaccggagcaacggtgcgcttcttccgcaccgtcatcccgctgcatctgccgcgcggcatcgacgcgtccatctcgttcgtgctgggcacgcctgccggcacgtccaccgcgtaccgcgcccagctgttcgtcaacggctaccagtacggccggtactacccgcacatcgggaaccaggtggtgtacccggttccggcgggagtgctggactacgacggtgagaacacgatcggcgtggcggtgtgggcgcagagtgacgccggggcggcgatcaatctggactggcgggtgaactacgttgccgacagctcgttggacgcggtgcggcttaccggggaggggtcgttaagaccccagtggagtgaggcaagagagcggtacgcttag

SEQ ID NO: 57 - protein, 1027 aa, Aspergillus carneus
MARLPQLLFLLLASVGLLSAAQNHTDSEWPLHDNGLNTVVQWDHYSFQVHGQRIFVFSGEFHYWRIPVPGLWRDILEKIKAAGFTAFAFYSSWAYHAPNNHTVDFSTGARDITPIYELAKELGMYIIVRPGPYVNAEASAGGYPLWVTTGAYGSLRNDDARYTEAWKPYFAKMSEITSQYQVTDGHNTFCYQIENEYGQQWIGDPVDRNPNQTAVAYMELLEESARENGIVVPLTANDPNMNTKSWGNDWSNAGGNVDVVGLDSYPSCWTCDVTQCTSTNGEYVPYKVMGYYDYFQEVQPTMPGFMPEFQGGSYNPWAGPEGGCPGDTGVDFANLFYRWNIAQRVTAMSLYMLYGGTNWGAIAAPVTATSYDYSSPISEDRSIGSKYYETKLLALFTRSATDLTMTDRIGNGTQYTNNPAVAAYELRNPVTNGAFYVTIHADSTVGSDESFRLNVNTSAGAFTVPSKGAIRLNGHQSKIVVTDFRFGPSHSLLYSTAEVLTHAVFDKQATIVLWVPTGESGEFAVKGAKSGKVESCPRCSNATFTRKKDVLVVNFTQTGGMSVLQLNNGVRVVLLDRPAAYNFWAPPVTDDPFAPETDLVLVQGPYLVRSASLSGSTLALRGDSIKETALEIFAPKKVKTVTWNGKRVKTSKSSYGSLTASLAPPPAVTLPALTSTRWKSQDSLPERLPSYDDSGPAWVDADHMTTQNPRTPETLPVLYADEYGFHNGIRLWRGSFTDAASGVYLNVQGGAAFGWSAYLNGHFLGSHLGTATTSQANKTLVFPTGALNQNATNTLLVIHDDTGHDQTTGALNPRGILAARLLPASNAAADSTAPTFTRWRVAGTAGGESDLDPVRGVYNEDGLFAERVGWHLPGFDDGAWPAANTTAVAQETGTVSLSFTGATVRFFRTVIPLHLPRGIDASISFVLGTPAGTSTAYRAQLFVNGYQYGRYYPHIGNQVVYPVPAGVLDYDGENTIGVAVWAQSDAGAAINLDWRVNYVADSSLDAVRLTGEGSLRPQWSEARERYA

SEQ ID NO: 58 - protein, 1007 aa, Aspergillus carneus
  REGION 1..1007: note = mat_peptide
AQNHTDSEWPLHDNGLNTVVQWDHYSFQVHGQRIFVFSGEFHYWRIPVPGLWRDILEKIKAAGFTAFAFYSSWAYHAPNNHTVDFSTGARDITPIYELAKELGMYIIVRPGPYVNAEASAGGYPLWVTTGAYGSLRNDDARYTEAWKPYFAKMSEITSQYQVTDGHNTFCYQIENEYGQQWIGDPVDRNPNQTAVAYMELLEESARENGIVVPLTANDPNMNTKSWGNDWSNAGGNVDVVGLDSYPSCWTCDVTQCTSTNGEYVPYKVMGYYDYFQEVQPTMPGFMPEFQGGSYNPWAGPEGGCPGDTGVDFANLFYRWNIAQRVTAMSLYMLYGGTNWGAIAAPVTATSYDYSSPISEDRSIGSKYYETKLLALFTRSATDLTMTDRIGNGTQYTNNPAVAAYELRNPVTNGAFYVTIHADSTVGSDESFRLNVNTSAGAFTVPSKGAIRLNGHQSKIVVTDFRFGPSHSLLYSTAEVLTHAVFDKQATIVLWVPTGESGEFAVKGAKSGKVESCPRCSNATFTRKKDVLVVNFTQTGGMSVLQLNNGVRVVLLDRPAAYNFWAPPVTDDPFAPETDLVLVQGPYLVRSASLSGSTLALRGDSIKETALEIFAPKKVKTVTWNGKRVKTSKSSYGSLTASLAPPPAVTLPALTSTRWKSQDSLPERLPSYDDSGPAWVDADHMTTQNPRTPETLPVLYADEYGFHNGIRLWRGSFTDAASGVYLNVQGGAAFGWSAYLNGHFLGSHLGTATTSQANKTLVFPTGALNQNATNTLLVIHDDTGHDQTTGALNPRGILAARLLPASNAAADSTAPTFTRWRVAGTAGGESDLDPVRGVYNEDGLFAERVGWHLPGFDDGAWPAANTTAVAQETGTVSLSFTGATVRFFRTVIPLHLPRGIDASISFVLGTPAGTSTAYRAQLFVNGYQYGRYYPHIGNQVVYPVPAGVLDYDGENTIGVAVWAQSDAGAAINLDWRVNYVADSSLDAVRLTGEGSLRPQWSEARERYA

SEQ ID NO: 59 - DNA, 3317 bp, Penicillium quercetorum
  sig_peptide 1..69
  mat_peptide 70..3314
  source 1..3317: mol_type = genomic DNA
  CDS 1..810
  CDS 876..1869
  CDS 1923..2216
  CDS 2273..2344
  CDS 2400..2487
  CDS 2540..3314
atgacgcgggcaacgcgtctattctacggattgggcacgatcttctccctgctcggtgctacaattgccgcggagaaccaaacaactaccgaatggcccctgcacgatgatggtctgaaccaagtcgtccaatgggaccactacagcttccagatcaacagtcagcgcatcttcatcttctcgggtgaattccactactggcgcatccccgttcctggtctgtggcgcgatatcctcgagaagatcaaggcggtgggtttcacggcgtttgccttttactcgagctgggcctaccatgcgcccaacaaccagacgctggactttaccaccggcgcgcatgactttactcccctgtttgagttggcgaaggagcttggactgtacattattgttcgccctggaccgtatgtcaatgccgaagccagtgcgggtggcttcccgctgtggctgactacgggtgattatggtacgcttcgcaataatgatacgcgctatacgaaagcctggacgccgtacttcaccaagatgtcccagatcaccagcaagtaccaggtcactgatgggcagaacgcgattgtctatcagatcgagaacgagtacggggagcaatgggttggctcggcgtcgaagcgtgtgcccaatgaaaaggctatcaactatatggaacttctcgaggccaatgcccgtgccaatggtattactgtgccattgactgcaaacgatccgaacatgaactcgcactcgtggggaagtgattggtctaaggagggtggtaatgtggatgttgcgggagtagactcgtacccttcggtaagttcgctcatgtttgctttaaatcatgactctggaagactgatgagcctgaatgaaaatagtgctggacctgcgacctcagccaatgtacctccaccaatggcgaatacatcccgttccaggtcatggactactacgattacttccaagagtcgcagccaaccatgcccgaattcatgcccgagttccagggtggttcatacaacccctggggtggtcctgaaggcggctgtgccgagaactcgaaccaggactttgcgaatctgttctaccggtggaacattggccaacgtgtcacagcgatgagcttatacatgctgttcggaggcacgaactggggtgcgattgcggcgcccgtcactggcagcagctacgattactcggctcctatctcagaggatcgatctatcggggacaagtactacgagaccaagctgctagctttgttcacgcgctgtgcgaaggacttgacgatgacgaacttgattggtaatgggactcagtatactgataatggcaatgtccgtgcctatgaactgcggaacccagacacgaacgccggtttctatgcgactttccacactaacacgtccgtctctaccaatgaagccttccatctcaaggtgaacacctctgctggtgccttgactgttcccacacatggcggtgtggttcgattgaacggacaccaatccaagattctggtgacggatttcacctttggaaaggagacgttgctgtattccaccgccgaggttttgacatatgccgtgtttgataagactcccacgctggttctgtggatgccgacgggtgaaacgggcgagttcaatatcaagggcgcaaagaagggatcggtccagaagtgtcagggatgctctagtgtgaagttcttcaaggagcacggcggtctgactgccgccattacccagtcttctggcatgagtgtgctggcgattgacgacatccaagtgattgtccttgacagaacatctgcgtataaattctgggctccggcgcttacgaatgacccgcttgtgcccgagacggagagtggtaagttacactacttgtagcgacttttcataccaaatctaaccatctggcagtgcttgttcaaggaccttatctcgttcgcggcgcttctctctcgggctcgaagcttgctgttacaggtgatattatcaacgctacgacactggaggtctttgccccgaaggctgttaagtctattacttggaatggaaagacccttaaaactcaacgtaccgagtatggtagtctgaaggggtccattgcggcacccaaggctgttactctaccctctttcaaatcctggaagtccaaagacagtcttcctgagcgtttggctgactatgatgatgcgggagctgcgtgggttggtaagaattgcctgttcttgacacacagcctatcattcatctaactgtccttctagatgcaaaccaccagtccacattgaaccctcgtgcccctactactctgccagtcatgtacgcagatgaatacggtaagcgctcccttcaatgcacacgtctagccaataatctgacagccatatccaggcttccacaacggcgtccgcctgtggcgcggatacttcaacggctctgcaacaggggcctacatcaacgtccagggtggatatgccttgtaagtccctctactcgaaccccaacccatgcccagcactaacacaatccagcggctggtccgcctggctcaacggccaattcatcggctcctacctcggctccgccgacctcgagtccggcaacctatccctatccttcaccaacgcaaccatcaacaccaacaaacccaacatcctcctcatcgtccatgacgacacaggccacgacgagacaagcggcgccctcaatccccgcggtatcctcgacgcccacctcctcggctcatcatccggcttcacccactggcgtctcgccggtaccgcgggcggcgagtccaacctcgaccccgtgcgcggcgtcttcaacgaagatgggctctacggcgaacgggttggctggcatctcccgggctacgacgactcgacctggtccagcagcggtggttcaagtctaagcttcactggcgcaacagtccgcttcttccgcacaaccatcccgctcaatttcccctccaacacagacgtatcaatctccttcatcttgtccacaccgtctggcagcacgaccgcataccgggcccagatctttgtgaacgggtaccagtacggccggtataacccgtacatcgggaaccaggtggtgtatcctgttccggcggggattttgaactacagcggggagaatacggtggctgttgctgtgtgggcgcagacggaggagggggcgaggatggaggtggattggcgggtgaattatgtggcggatagttcgttggatgttgttagtgttagtaagaaggcggaggggttgaggacgaagtggactgaggtgcgggagaagtttgcttga

SEQ ID NO: 60 - protein, 1011 aa, Penicillium quercetorum
MTRATRLFYGLGTIFSLLGATIAAENQTTTEWPLHDDGLNQVVQWDHYSFQINSQRIFIFSGEFHYWRIPVPGLWRDILEKIKAVGFTAFAFYSSWAYHAPNNQTLDFTTGAHDFTPLFELAKELGLYIIVRPGPYVNAEASAGGFPLWLTTGDYGTLRNNDTRYTKAWTPYFTKMSQITSKYQVTDGQNAIVYQIENEYGEQWVGSASKRVPNEKAINYMELLEANARANGITVPLTANDPNMNSHSWGSDWSKEGGNVDVAGVDSYPSCWTCDLSQCTSTNGEYIPFQVMDYYDYFQESQPTMPEFMPEFQGGSYNPWGGPEGGCAENSNQDFANLFYRWNIGQRVTAMSLYMLFGGTNWGAIAAPVTGSSYDYSAPISEDRSIGDKYYETKLLALFTRCAKDLTMTNLIGNGTQYTDNGNVRAYELRNPDTNAGFYATFHTNTSVSTNEAFHLKVNTSAGALTVPTHGGVVRLNGHQSKILVTDFTFGKETLLYSTAEVLTYAVFDKTPTLVLWMPTGETGEFNIKGAKKGSVQKCQGCSSVKFFKEHGGLTAAITQSSGMSVLAIDDIQVIVLDRTSAYKFWAPALTNDPLVPETESVLVQGPYLVRGASLSGSKLAVTGDIINATTLEVFAPKAVKSITWNGKTLKTQRTEYGSLKGSIAAPKAVTLPSFKSWKSKDSLPERLADYDDAGAAWVDANHQSTLNPRAPTTLPVMYADEYGFHNGVRLWRGYFNGSATGAYINVQGGYAFGWSAWLNGQFIGSYLGSADLESGNLSLSFTNATINTNKPNILLIVHDDTGHDETSGALNPRGILDAHLLGSSSGFTHWRLAGTAGGESNLDPVRGVFNEDGLYGERVGWHLPGYDDSTWSSSGGSSLSFTGATVRFFRTTIPLNFPSNTDVSISFILSTPSGSTTAYRAQIFVNGYQYGRYNPYIGNQVVYPVPAGILNYSGENTVAVAVWAQTEEGARMEVDWRVNYVADSSLDVVSVSKKAEGLRTKWTEVREKFA

SEQ ID NO: 61 - protein, 988 aa, Penicillium quercetorum
  REGION 1..988: note = mat_peptide
AENQTTTEWPLHDDGLNQVVQWDHYSFQINSQRIFIFSGEFHYWRIPVPGLWRDILEKIKAVGFTAFAFYSSWAYHAPNNQTLDFTTGAHDFTPLFELAKELGLYIIVRPGPYVNAEASAGGFPLWLTTGDYGTLRNNDTRYTKAWTPYFTKMSQITSKYQVTDGQNAIVYQIENEYGEQWVGSASKRVPNEKAINYMELLEANARANGITVPLTANDPNMNSHSWGSDWSKEGGNVDVAGVDSYPSCWTCDLSQCTSTNGEYIPFQVMDYYDYFQESQPTMPEFMPEFQGGSYNPWGGPEGGCAENSNQDFANLFYRWNIGQRVTAMSLYMLFGGTNWGAIAAPVTGSSYDYSAPISEDRSIGDKYYETKLLALFTRCAKDLTMTNLIGNGTQYTDNGNVRAYELRNPDTNAGFYATFHTNTSVSTNEAFHLKVNTSAGALTVPTHGGVVRLNGHQSKILVTDFTFGKETLLYSTAEVLTYAVFDKTPTLVLWMPTGETGEFNIKGAKKGSVQKCQGCSSVKFFKEHGGLTAAITQSSGMSVLAIDDIQVIVLDRTSAYKFWAPALTNDPLVPETESVLVQGPYLVRGASLSGSKLAVTGDIINATTLEVFAPKAVKSITWNGKTLKTQRTEYGSLKGSIAAPKAVTLPSFKSWKSKDSLPERLADYDDAGAAWVDANHQSTLNPRAPTTLPVMYADEYGFHNGVRLWRGYFNGSATGAYINVQGGYAFGWSAWLNGQFIGSYLGSADLESGNLSLSFTNATINTNKPNILLIVHDDTGHDETSGALNPRGILDAHLLGSSSGFTHWRLAGTAGGESNLDPVRGVFNEDGLYGERVGWHLPGYDDSTWSSSGGSSLSFTGATVRFFRTTIPLNFPSNTDVSISFILSTPSGSTTAYRAQIFVNGYQYGRYNPYIGNQVVYPVPAGILNYSGENTVAVAVWAQTEEGARMEVDWRVNYVADSSLDVVSVSKKAEGLRTKWTEVREKFA

SEQ ID NO: 62 - protein, 331 aa, Humicola insolens
  REGION 1..331: note = mat_peptide
LQYKGVDWSSVMVEERAGVRYKNVNGQEKPLEYILAENGVNMVRQRVWVNPWDGNYNLDYNIQLARRAKAAGLGLYINFHYSDTWADPAHQTTPAGWPSDINNLAWKLYNYTLDSMNRFADAGIQVDIVSIGNEITQGLLWPLGKTNNWYNIARLLHSAAWGVKDSRLNPKPKIMVHLDNGWNWDTQNWWYTNVLSQGPFEMSDFDMMGVSFYPFYSASATLDSLRRSLNNMVSRWGKEVAVVETNWPTSCPYPRYQFPADVRNVPFSAAGQTQYIQSVANVVSSVSKGVGLFYWEPAWIHNANLGSSCADNTMFTPSGQALSSLSVFHRI

SEQ ID NO: 63 - protein, 332 aa, Myceliophthora thermophile
  REGION 1..332: note = mat_peptide
ALTYRGVDWSSVVVEERAGVSYKNTNGNAQPLENILAANGVNTVRQRVWVNPADGNYNLDYNIAIAKRAKAAGLGVYIDFHYSDTWADPAHQTMPAGWPSDIDNLSWKLYNYTLDAANKLQNAGIQPTIVSIGNEIRAGLLWPTGRTENWANIARLLHSAAWGIKDSSLSPKPKIMIHLDNGWDWGTQNWWYTNVLKQGTLELSDFDMMGVSFYPFYSSSATLSALKSSLDNMAKTWNKEIAVVETNWPISCPNPRYSFPSDVKNIPFSPEGQTTFITNVANIVSSVSRGVGLFYWEPAWIHNANLGSSCADNTMFSQSGQALSSLSVFQRI

SEQ ID NO: 64 - protein, 324 aa, Meripilus giganteus
  REGION 1..324: note = mat_peptide
LTYKGADISSVPLVEQAGIKYTDGGKVTPFENIIHNHGANTVRIRIWTAGDYNLQYGLALAKRVKAAGLTLVVDLHYSDTWADPGKQAIPSAWPKDLDGLNTQIWQYTKDVVTSFANQGTPIDILQVGNEINNGLLWPVGEISSNGINPVSQLLHSAINGAKAAGNPKILIHLANGWDWSGLNSFFGKVFIPGALSADEVDIIGVSFYPFYDAGATLSALKSSLANLANTFKKPIVVAETDWPVACSGVKLTEPSVPVSTSGQQTWIGDIKNVLQSLPNGLGQGIFYWEPGWIGNANLGSGCSDNLLVSSNGATRDSINIFNQM

SEQ ID NO: 65 - protein, 12 aa, synthetic construct
  REGION 1..12: note = SEQ ID NO: 65 is the conserved motif GV[T/M]PD[W/M]VQ[I/V]GNE.
  SITE 3: note = misc_feature - The amino acid in position 3 of the conserved motif is either threonine (T) or methionine (M).
  SITE 6: note = misc_feature - The amino acid in position 6 of the conserved motif is either tryptophan (W) or methionine (M).
  SITE 9: note = misc_feature - The amino acid in position 9 of the conserved motif is either isoleucine (I) or valine (V).
GVXPDXVQXGNE

SEQ ID NO: 66 - protein, 13 aa, synthetic construct
  REGION 1..13: note = SEQ ID NO: 66 is the conserved motif WADP[A/G]xQxKPxAW.
  SITE 5: note = misc_feature - The amino acid in position 5 of the conserved motif is either alanine (A) or glycine (G).
  SITE 6: note = misc_feature - The amino acid in position 6 of the conserved motif is any amino acid.
  SITE 8: note = misc_feature - The amino acid in position 8 of the conserved motif is any amino acid.
  SITE 11: note = misc_feature - The amino acid in position 11 of the conserved motif is any amino acid.
WADPXXQXKPXAW

SEQ ID NO: 67 - protein, 27 aa, Bacillus clausii
MKKPLGKIVASTALLISVAFSSSIASA

SEQ ID NO: 68 - DNA, 3138 bp, Penicillium simplicissimum
  sig_peptide 1..63
  mat_peptide 64..3135
  source 1..3138: mol_type = genomic DNA
  CDS 1..235
  CDS 306..1382
  CDS 1439..1940
  CDS 2001..3135
atgcggtttttcgcatttctcccgttgctccttatcggggcgctgtcgagcattgtctctgcgacggacaatggcaagactaccgatgttacttgggacaagtatagtctctccgtgaagggggagagagtctttgtcttttctggtgaattccattatatgcgtcttcctgttccggagatgtggcttgatgtgttccaaaagttgcgctccaatggcttcaacgcggtatccagtgagtaaaccaatatatatcccatacaccacactcaatcaattaaaaccaattcaactaaccgttcaagtctacttcttctggagcttccactccgcttcggaagacacatttgactttgaaaacggcgcccacgatgtccagcgcgtcttcgactacgctaaacaagccggtctgtatgtgattgcccgtgcaggaccctacatcaacgctgaaacctcggccggtggattcgccctgtgggcagcgaacggacaaatgggcagtgaacgaaccagtgcctcgtcctactacgacaaatggcttccctggatcctgaagatcggcaagatcatcgcggataaccagatcaccaacggcggaccggtgatcctgaaccagcacgagaacgagctccaggagaccacccacagcgcgaccaacactctagttctgtacatggagcaaatcgcagccgcattcgaggaggccggtgtcatcgtgcccagctcgcacaacgaaaaaggtatgcgctcggaaagctggtcgacagattacgaagacgtcggcggtgcagtaaacgtctacggcctcgattcataccccggcggtctgtcctgcacaaaccccgactcgggattcaacctcgtccgcacttactaccaatggttccagaactactcctacacacagcccgaattcctccccgaatttgagggcggctggttccagccctggggtggatatttctacgacgagtgtgccgcagagcactcgcccgaattcgccgacgtctattacaagaataacattgggtcccgggtcaccctgcagagtctgtatatggcctttggcgggacgaattggggtcatagtgccacgccggtcgtttatacttcgtatgactatgcggcgccgctaagggagacgagagagatccaggataaactcaagcagactaagttgattggtttgtttactcgggtttcatcgggattgttgcagactgtcatggagggcaatggaacgggatatactagtgatactagtatttatacgtgggctttgcggaatcccgagacggacgctgggttctatgtgcttgcgcatagtacgagttcgtctcgtgcggtgacgacgttctcgctgaatgttaatacttcggctggtatggttcctcacgctggagtgctttgagaatattttgactaactcgcttcttaggtgctctgactatccctgacattgaactggatggtcgccaaagcaaaatcatcgtcacggattacgaaatcggcaaggcctcgagccttctctactcatccgccgaggttctgacctacgctaccctcgacgtggacgtgctggtgctctacctgaacattggacaaaagggcgtgttcgcattcaagaatgccccatcccacttgacgttcaagacatacggtaactcgaacttgacttccaccacatcgaccaatggaacgcagtactcgtacacccaaggagatggtgcgaccgctgtcaagttctccaacggggttcttctatatctgctggacaaggaaaccgcttggaacttctttgctgtgactaccacgtccaacccgaatgtgacccccagcgaacacattcttgctcttggaccgtatttggttcgtgaggcgagtatcagccatgataccgttagcctgattggtgataatgcgaataccaccacactggagtaagttgattcccatggaagggtatttggtggaactgcacttgctaacctttctcatagagtctaccctggtaacgcccaggtaaccaagatcaagtggaatggcaaaccgattgcgactaagaagaccgcatacggcagtctcatcggctcagcccaaggcgcagaaaccgccaagatctccctgccctctctgacatcctggaagtctcaagatactcttcccgagatcaagcaagactacgacgactcgcgctggacggtctgcaacaagagcacgacggtcaactctgtcgcaccactgtcgctgcccgtcctatactcgggcgactacggataccacgcaggcaccaagatctaccgcggtcgcttcgacggacgcaatgccaccggcgccaacgtgacggtgcaaaacggcgtcgccgctggctgggcagcctggttgaacggcgactatgttggcggtgccctaggcaatccagctctcgcagcaacctccgacttgttaaccttcaacagctcctccctccgggataccgataacgtcctcacggtcgtgatggactataccggccacgacgagaacaacgtcaagccggccggtacccagaacccccgcggtatcttgggagccaccctcttcggcggcggcaacttcacctcctggcgcatccaaggcaacgcaggcggcgaagcaaacatcgaccccgtccgcggccccatgaacgaaggtggcctctacggcgaacgactcggctggcatctcccgggatacaccgcacccaagagcgcgggcagctcatcccccctgcagggtgtctcgaacgccgcaggacgcttctacacgacaaccttcaagctcaatctagaggccgatctggacgtcccgattggcctgcagctcggggcagcggccaataccagtgcggtggtgcaggtgtttatgaacgggtaccagtttggccattacctgccgcatattggaccgcagacgctgttcccgttcccaccgggtattatcaataatcggggggagaatacgttggcgattagtctgtgggcgttgacggatgagggggcggcgttggatcaggtggagttggtcgcgtacggggcgtatcggaccgggttcgattttaatcaggattggacgtacctgcagccgaagtggaagaataatcgggggtcgtatgtgtag

SEQ ID NO: 69 - protein, 983 aa, Penicillium simplicissimum
MRFFAFLPLLLIGALSSIVSATDNGKTTDVTWDKYSLSVKGERVFVFSGEFHYMRLPVPEMWLDVFQKLRSNGFNAVSIYFFWSFHSASEDTFDFENGAHDVQRVFDYAKQAGLYVIARAGPYINAETSAGGFALWAANGQMGSERTSASSYYDKWLPWILKIGKIIADNQITNGGPVILNQHENELQETTHSATNTLVLYMEQIAAAFEEAGVIVPSSHNEKGMRSESWSTDYEDVGGAVNVYGLDSYPGGLSCTNPDSGFNLVRTYYQWFQNYSYTQPEFLPEFEGGWFQPWGGYFYDECAAEHSPEFADVYYKNNIGSRVTLQSLYMAFGGTNWGHSATPVVYTSYDYAAPLRETREIQDKLKQTKLIGLFTRVSSGLLQTVMEGNGTGYTSDTSIYTWALRNPETDAGFYVLAHSTSSSRAVTTFSLNVNTSAGALTIPDIELDGRQSKIIVTDYEIGKASSLLYSSAEVLTYATLDVDVLVLYLNIGQKGVFAFKNAPSHLTFKTYGNSNLTSTTSTNGTQYSYTQGDGATAVKFSNGVLLYLLDKETAWNFFAVTTTSNPNVTPSEHILALGPYLVREASISHDTVSLIGDNANTTTLEVYPGNAQVTKIKWNGKPIATKKTAYGSLIGSAQGAETAKISLPSLTSWKSQDTLPEIKQDYDDSRWTVCNKSTTVNSVAPLSLPVLYSGDYGYHAGTKIYRGRFDGRNATGANVTVQNGVAAGWAAWLNGDYVGGALGNPALAATSDLLTFNSSSLRDTDNVLTVVMDYTGHDENNVKPAGTQNPRGILGATLFGGGNFTSWRIQGNAGGEANIDPVRGPMNEGGLYGERLGWHLPGYTAPKSAGSSSPLQGVSNAAGRFYTTTFKLNLEADLDVPIGLQLGAAANTSAVVQVFMNGYQFGHYLPHIGPQTLFPFPPGIINNRGENTLAISLWALTDEGAALDQVELVAYGAYRTGFDFNQDWTYLQPKWKNNRGSYV

SEQ ID NO: 70 - protein, 962 aa, Penicillium simplicissimum
  REGION 1..962: note = mat_peptide
TDNGKTTDVTWDKYSLSVKGERVFVFSGEFHYMRLPVPEMWLDVFQKLRSNGFNAVSIYFFWSFHSASEDTFDFENGAHDVQRVFDYAKQAGLYVIARAGPYINAETSAGGFALWAANGQMGSERTSASSYYDKWLPWILKIGKIIADNQITNGGPVILNQHENELQETTHSATNTLVLYMEQIAAAFEEAGVIVPSSHNEKGMRSESWSTDYEDVGGAVNVYGLDSYPGGLSCTNPDSGFNLVRTYYQWFQNYSYTQPEFLPEFEGGWFQPWGGYFYDECAAEHSPEFADVYYKNNIGSRVTLQSLYMAFGGTNWGHSATPVVYTSYDYAAPLRETREIQDKLKQTKLIGLFTRVSSGLLQTVMEGNGTGYTSDTSIYTWALRNPETDAGFYVLAHSTSSSRAVTTFSLNVNTSAGALTIPDIELDGRQSKIIVTDYEIGKASSLLYSSAEVLTYATLDVDVLVLYLNIGQKGVFAFKNAPSHLTFKTYGNSNLTSTTSTNGTQYSYTQGDGATAVKFSNGVLLYLLDKETAWNFFAVTTTSNPNVTPSEHILALGPYLVREASISHDTVSLIGDNANTTTLEVYPGNAQVTKIKWNGKPIATKKTAYGSLIGSAQGAETAKISLPSLTSWKSQDTLPEIKQDYDDSRWTVCNKSTTVNSVAPLSLPVLYSGDYGYHAGTKIYRGRFDGRNATGANVTVQNGVAAGWAAWLNGDYVGGALGNPALAATSDLLTFNSSSLRDTDNVLTVVMDYTGHDENNVKPAGTQNPRGILGATLFGGGNFTSWRIQGNAGGEANIDPVRGPMNEGGLYGERLGWHLPGYTAPKSAGSSSPLQGVSNAAGRFYTTTFKLNLEADLDVPIGLQLGAAANTSAVVQVFMNGYQFGHYLPHIGPQTLFPFPPGIINNRGENTLAISLWALTDEGAALDQVELVAYGAYRTGFDFNQDWTYLQPKWKNNRGSYV

SEQ ID NO: 71 - DNA, 3309 bp, Aspergillus westerdijkiae
  sig_peptide 1..60
  mat_peptide 61..3306
  source 1..3309: mol_type = genomic DNA
  CDS 1..801
  CDS 852..1848
  CDS 1898..2191
  CDS 2239..2310
  CDS 2360..2447
  CDS 2499..3306
atggcgcgcatcatgcaccttgccgtgctgcttctttccagcatcggactgctggctgctgcccagaatcagtccgactctgactggcctctgcacgacaacggtctgaacaccgccgtgcaatgggaccattacagcttccatgtccacggacagcgcatcttcatcttctccggcgagtttcactactggcgtattcccgtccccgagctttggcgcgacatcctcgagaaggtcaaagccaccggcttcaccgcgtttgccttctactctagctgggcgtaccatgcgccgaacaaccacacggtggacttccacaccggtgcgcgcgacatcacgcccatcttcgagctcgccaaggagctgggcatgtatatgatcgtgcggcccgggccgtatgtcaatgccgaggccagcgctggtggctttccgctgtgggcgaccaccggtgcgtatgggtcgatgcgcaatgacgaccccaggtatactgcggcgtggaagccgtactttgagaagatgtcgcaaatcaccagtcagtaccagatcaccgatggggaaaacactttctgctatcagatcgagaacgagtatggccagcagtgggttggtgatccccgtgatcggaacccgaataagactgcggtcgcctatatggaactgctcgaggagagtgcccgtgagaatggtattgtcgtgccgctgacggccaacgatccgaacctgaacacccgctcttggggaaacgactggtccaacgctggaggaaacgttgacgttcctggagtggattcgtatccctcagtgagttacctaaatcacatctgggtaatgcaaattactaatctttccagtgctggacttgtgatgtctctcaatgcacctccaccaacggagagtacgttccttacaaagtgatcccctattacgactacttccaggaggtccagccctcgatgcctgccttcatgcccgaattccagggtggatcttacaacccctgggccggccccgaaggtggatgtcccgaggataccggagcggactttgccaacctgttctaccggtggaacatcgcccagcgagtgaccgccatgagcttgtacatggtatttggcggaaccaactggggctcgctggctgcccccgttacagccaccagctacgactactcctccccgattgccgaagaccgctcgattggtgacaagtactacgagaccaagctgctttccctgttcactcgtagcgccaaggatctcaccatgaccgacctcatcggcaacggcaccaagtacaccgacaatgctgccgtcagcgcgtacgaactccggaaccccgagaccaacggtgccttctacgtcaccatccacaaggacaccaccgtcggctcggacgagtccttcaagctccacgtgaacacctccgctggcgcgctgactatcccaagcgagggggcaaagatccgcctgaacggccatcagtccaagatcatcgtgactgactttgccttcggctctaagaccctcctgtactccaccgccgaggtgttgacctatgcggtcatcgatgaccagcctactctggtgctttgggtcccgaagggagaatctggcgagttcgctgtcaagggcactaagtctggcaaggtggcgagctgcaacggctgctccagcgtcaagttcaacggaaagaaggaccacgtggttgttgggttcacacaggccaagggcatgagcgtgtatcagctggatgatgatgtccgtgtcgttgttctcgaccggtcgtccgcttatcacttctgggcccctactttgactgatgatccgattgccccggaggatgaaattggtatgctcccgtgtccgagagaaatgactgattgctaatatcatactagtcctggtcgagggcccctacctcgtccgctcggccagcgtcgagggatctacccttgctctccgcggtgactctaccgacaagaccaacctggaggttttcgctcctaagagcgtcaagaccatcacctggaatggcaagaaggtcaagtcctccgagacctcctatggcagcctcaaggccacgctcgccgcgccaccctcgattaagctaccctctttcggctcatggcggtcgaacgacagcttgccggagcgcttggagtcgtacgatgactctggcccggcctgggttggtaagtacatctccacggcggtccaagattcccgctcaccagaacagatgccaaccatgaaaccacgctgaacccgcatccccctgtcacgactcctgtcttgtacgcaaacgaatacggtatgcatctctggccttcattctttagtctcatgctcatcacgtccaggcttccacaacggcgtccgcctctggcgcggctatttcaacggaaccgcctccggcgtcttcctcaacatccaaggtggcgctgcattgtaagcaccctctccctcctaacatccacgaccatctaaccaaaagtccagcggctggtccgcctatctcaacggccacttccttggctcctacctcggcaacgccaccatcgcgcaagccaacaaaaccctcaccttcccgaacaacacgctccacacgcgccccggctcccggaacaccctcctcgtcatccacgacgacaccggccacgaccagaccaccggcgtgctcaacccgcgcggcatcatcgaagcccgcctcctcggctccaacgccccgaacttcacccactggcgtctcgccggtaccgccggcggcgaatcaaacctcgatcccgtccgcggcgtctacaacgaagacggcctccacgcggagcgcgtcggctggcatctccctggcttcgacgacagcgactggcctgtcaccaaccactcctcctcctcctctagctccaaatccctctccaccctctccttcaccggcgcaaccgttcgcttcttccgcaccaccatccccctaaatatcccctcgggcctcgacgtctcgatctccttcctcctcggcacgccgacaggcacgagtaaggcctaccgcgcgcagctcttcgttaacggctaccagtacgggcgctactatccgcacatcggcaaccaggtcgtgtatccggtcccggcggggattttggattaccgcggcgagaacacgatcgggttggctgtttgggcgcagagcgaggatggcgcggcggtcagtgttgattggagggtgaattatgtggcggatagttcgttggatgttgcggggattggggaggagaggttgaggccggggtatgagaaggtgagggagaagtttgcttga

SEQ ID NO: 72 - protein, 1020 aa, Aspergillus westerdijkiae
MARIMHLAVLLLSSIGLLAAAQNQSDSDWPLHDNGLNTAVQWDHYSFHVHGQRIFIFSGEFHYWRIPVPELWRDILEKVKATGFTAFAFYSSWAYHAPNNHTVDFHTGARDITPIFELAKELGMYMIVRPGPYVNAEASAGGFPLWATTGAYGSMRNDDPRYTAAWKPYFEKMSQITSQYQITDGENTFCYQIENEYGQQWVGDPRDRNPNKTAVAYMELLEESARENGIVVPLTANDPNLNTRSWGNDWSNAGGNVDVPGVDSYPSCWTCDVSQCTSTNGEYVPYKVIPYYDYFQEVQPSMPAFMPEFQGGSYNPWAGPEGGCPEDTGADFANLFYRWNIAQRVTAMSLYMVFGGTNWGSLAAPVTATSYDYSSPIAEDRSIGDKYYETKLLSLFTRSAKDLTMTDLIGNGTKYTDNAAVSAYELRNPETNGAFYVTIHKDTTVGSDESFKLHVNTSAGALTIPSEGAKIRLNGHQSKIIVTDFAFGSKTLLYSTAEVLTYAVIDDQPTLVLWVPKGESGEFAVKGTKSGKVASCNGCSSVKFNGKKDHVVVGFTQAKGMSVYQLDDDVRVVVLDRSSAYHFWAPTLTDDPIAPEDEIVLVEGPYLVRSASVEGSTLALRGDSTDKTNLEVFAPKSVKTITWNGKKVKSSETSYGSLKATLAAPPSIKLPSFGSWRSNDSLPERLESYDDSGPAWVDANHETTLNPHPPVTTPVLYANEYGFHNGVRLWRGYFNGTASGVFLNIQGGAAFGWSAYLNGHFLGSYLGNATIAQANKTLTFPNNTLHTRPGSRNTLLVIHDDTGHDQTTGVLNPRGIIEARLLGSNAPNFTHWRLAGTAGGESNLDPVRGVYNEDGLHAERVGWHLPGFDDSDWPVTNHSSSSSSSKSLSTLSFTGATVRFFRTTIPLNIPSGLDVSISFLLGTPTGTSKAYRAQLFVNGYQYGRYYPHIGNQVVYPVPAGILDYRGENTIGLAVWAQSEDGAAVSVDWRVNYVADSSLDVAGIGEERLRPGYEKVREKFA

SEQ ID NO: 73 - protein, 1000 aa, Aspergillus westerdijkiae
  REGION 1..1000: note = mat_peptide
AQNQSDSDWPLHDNGLNTAVQWDHYSFHVHGQRIFIFSGEFHYWRIPVPELWRDILEKVKATGFTAFAFYSSWAYHAPNNHTVDFHTGARDITPIFELAKELGMYMIVRPGPYVNAEASAGGFPLWATTGAYGSMRNDDPRYTAAWKPYFEKMSQITSQYQITDGENTFCYQIENEYGQQWVGDPRDRNPNKTAVAYMELLEESARENGIVVPLTANDPNLNTRSWGNDWSNAGGNVDVPGVDSYPSCWTCDVSQCTSTNGEYVPYKVIPYYDYFQEVQPSMPAFMPEFQGGSYNPWAGPEGGCPEDTGADFANLFYRWNIAQRVTAMSLYMVFGGTNWGSLAAPVTATSYDYSSPIAEDRSIGDKYYETKLLSLFTRSAKDLTMTDLIGNGTKYTDNAAVSAYELRNPETNGAFYVTIHKDTTVGSDESFKLHVNTSAGALTIPSEGAKIRLNGHQSKIIVTDFAFGSKTLLYSTAEVLTYAVIDDQPTLVLWVPKGESGEFAVKGTKSGKVASCNGCSSVKFNGKKDHVVVGFTQAKGMSVYQLDDDVRVVVLDRSSAYHFWAPTLTDDPIAPEDEIVLVEGPYLVRSASVEGSTLALRGDSTDKTNLEVFAPKSVKTITWNGKKVKSSETSYGSLKATLAAPPSIKLPSFGSWRSNDSLPERLESYDDSGPAWVDANHETTLNPHPPVTTPVLYANEYGFHNGVRLWRGYFNGTASGVFLNIQGGAAFGWSAYLNGHFLGSYLGNATIAQANKTLTFPNNTLHTRPGSRNTLLVIHDDTGHDQTTGVLNPRGIIEARLLGSNAPNFTHWRLAGTAGGESNLDPVRGVYNEDGLHAERVGWHLPGFDDSDWPVTNHSSSSSSSKSLSTLSFTGATVRFFRTTIPLNIPSGLDVSISFLLGTPTGTSKAYRAQLFVNGYQYGRYYPHIGNQVVYPVPAGILDYRGENTIGLAVWAQSEDGAAVSVDWRVNYVADSSLDVAGIGEERLRPGYEKVREKFA

SEQ ID NO: 74 - DNA, 3299 bp, Aspergillus wentii
  sig_peptide 1..60
  mat_peptide 61..3296
  source 1..3299: mol_type = genomic DNA
  CDS 1..789
  CDS 836..1829
  CDS 1877..2170
  CDS 2220..2291
  CDS 2339..2426
  CDS 2474..3296
atggcgcgcattttccatttgtttcttgccctactttcaagtatagggcttttggcagctgcagagtcacaatggcctctccacgataacagcttaaacaccgtcgttcaatgggatcattacagcttccagatccacgggcagagaatcttcgtcttctccggtgaattccactactggcgcattccagttccaggactatggagggatattcttgagaagattaaagcggctggatttactgcattcgcattttactccagttgggcttaccatgcgccaaataaccataccgttgacttttcgaccggtgctcgtgatatcacacctattttcgaacttgccaaggagttgggcttgtatatcatcgttcgcccagggccatatgtcaatgcggaagccaatgctggtggctttcccttgtggctgacgactggggaatacggaacgctacgcaatgacgatgaacgctatactgccgcgtggaagccgtacttcactaaaatgtcgcagattacgagcaaatatcagatcacggatggcgagaacaccttgttttatcagattgaaaacgaatacggagaccagtggatcggcgatccaagtgatcgagttccgaataatactgcaattgcttatatggagcttctcgaggcgagtgcacgggaaaacggcatcaatgtacctctcaccgcgaatgatcctaatatgaactcgaaatcttgggggaaagattggtctaatgctggtggaaacgttgacgcccctggcttggactcttacccgtcggtaggttaaccataactctaagactggattattctgacagtagcagtgttggacgtgtgatattagccaatgcacctcgacgaatggcgagtatgtgccgtacaaagtaatgcagtattacgactacttccaagaagttcaaccgacaacgccgtctttcatgcccgagttccagggcggttcttacaatccctgggcaggacctgaaggtggatgctccgagaataccggggcagactttgcgaatctgttctatcggtggaacattggccagcatgtgacggctatgagtctgtacatgctatacggaggtacgaattgggggtcgctcgctgcaccggtgacggcaagtagttatgactactcagccccgatttccgaagatcggtctattggggcaaagtattatgagactaaactactggcattgttcacgcggtgtgcaagagatttgaccatgactgaattgattggaaatggaactcagtataccgataatatagcagtggaagcatacgaattgaggaatccgcagaccaatgccggtttctacgttaccatccacagcaactcttcctctgggacaaacgaggcctttcaacttcaggtcaacacttctgtcggaggtctgactgttcctagccatggaggtactatacgtctcaatggtcaccagtccaagattatcgtgacggactttacatttggttccaagactcttctctattccaccgcggaggttctcacctacgctgtgttggatgacaaacctacacttgtcctctgggtacctaccggagaatccggcgagttctccatcaaaggagtcaagtctggatcagtcagtaactgtcagggctgctcgggtatgggtttctaccaggaaaatggtggtctcacggtaagattcacccagtcatctggaatgagcatcctccagctcgacgatgtacgcgtggttttactcgatagaacaagcgcatataatttctgggcgcctgcattgacaaatgacccatttgttccagagacagaaagtggtatgtttcgcctgatttattaattggcatttactaaccggtcgaagttctgattcaaggtccatacctcgttcgcggtgccaaaattactgaatcaactcttgcagtgactggtgattctgtggatgctacgagtatcgaggtcttcgcaccccagaccttggatacaatcacctggaatggcaaagaggtcaaaaccacgaggacggaatatggaagtctgcgggcttctcttgctgcaccaccatctattaagttaccctcgttgacatcgtggaaaacaaaagacagtctaccagagcggttgccatcatatgatgactctggtgaggcgtgggctggtaagtgccacttatctatctacactcactcaatgctaatcgaggatagatgccaaccatatgacaacttcgaatccacataaaccagaaacttatcccgttctttatggggatgattatggtatgtccattgtatccatgatagttatcaataagctaacaaagaaggcttccacaacggcatccgtctctggcgaggatactttaacaacaccgcgaaaggcgtctacctgaacatccaaggaggaacagctttgtaagatccatctcttttccatttaggtgaacaagctaacaaatcagtggctggtctgcctatctgaacggccacttcctctcctcttacctgggcaatgcaacagaaacccaaggaaataagaccatcctcttcccatctgatatcctctccacaaaaccagaaacgaatccaaataccctcctcatcatccacgatgacacaggccacgaccaaacaaccggcgttctcaacccgcgcggcatcctcgaagcacgtctcctcgacgaagacgagaaaagcagtgaagacctcgcatttacgcactggcgcgttgcaggtacagctggaggagaatcgaatctcgatcccgtccgcggcgtatacaatgaagacggactatacgccgaacggatgggctggcatttacccggtttcgacgatagtgattggtctacgattaacacaaccacgtccagtactaccagcagccccccattaacattcaccaacgcaaccatccaattcttccgaagcgtcatccccctcgacctccccaacaacaccgacacatccatgtccttcatcctctccactccatccaccagcagcaaagcctaccgcgcccaaatattcataaacgggtaccaatacggccggtacaacccccacatcgggaaccaggtggtcttccccgttccgccggggatactggattaccacggcgacaacacgattggagtagcggtgtgggcacagagcgaggatggggcgagtattgaattagattggagggtgaattacgttgctgatagttcgctggatgtgggccgtttggatgaggggggatcgctgaggccggggtggagtgaggagaggttgaggtttgcgtga

SEQ ID NO: 75 - protein, 1020 aa, Aspergillus wentii
MARIFHLFLALLSSIGLLAAAESQWPLHDNSLNTVVQWDHYSFQIHGQRIFVFSGEFHYWRIPVPGLWRDILEKIKAAGFTAFAFYSSWAYHAPNNHTVDFSTGARDITPIFELAKELGLYIIVRPGPYVNAEANAGGFPLWLTTGEYGTLRNDDERYTAAWKPYFTKMSQITSKYQITDGENTLFYQIENEYGDQWIGDPSDRVPNNTAIAYMELLEASARENGINVPLTANDPNMNSKSWGKDWSNAGGNVDAPGLDSYPSCWTCDISQCTSTNGEYVPYKVMQYYDYFQEVQPTTPSFMPEFQGGSYNPWAGPEGGCSENTGADFANLFYRWNIGQHVTAMSLYMLYGGTNWGSLAAPVTASSYDYSAPISEDRSIGAKYYETKLLALFTRCARDLTMTELIGNGTQYTDNIAVEAYELRNPQTNAGFYVTIHSNSSSGTNEAFQLQVNTSVGGLTVPSHGGTIRLNGHQSKIIVTDFTFGSKTLLYSTAEVLTYAVLDDKPTLVLWVPTGESGEFSIKGVKSGSVSNCQGCSGMGFYQENGGLTVRFTQSSGMSILQLDDVRVVLLDRTSAYNFWAPALTNDPFVPETESVLIQGPYLVRGAKITESTLAVTGDSVDATSIEVFAPQTLDTITWNGKEVKTTRTEYGSLRASLAAPPSIKLPSLTSWKTKDSLPERLPSYDDSGEAWADANHMTTSNPHKPETYPVLYGDDYGFHNGIRLWRGYFNNTAKGVYLNIQGGTAFGWSAYLNGHFLSSYLGNATETQGNKTILFPSDILSTKPETNPNTLLIIHDDTGHDQTTGVLNPRGILEARLLDEDEKSSEDLAFTHWRVAGTAGGESNLDPVRGVYNEDGLYAERMGWHLPGFDDSDWSTINTTTSSTTSSPPLTFTNATIQFFRSVIPLDLPNNTDTSMSFILSTPSTSSKAYRAQIFINGYQYGRYNPHIGNQVVFPVPPGILDYHGDNTIGVAVWAQSEDGASIELDWRVNYVADSSLDVGRLDEGGSLRPGWSEERLRFA

SEQ ID NO: 76 - protein, 1000 aa, Aspergillus wentii
  REGION 1..1000: note = mat_peptide
AESQWPLHDNSLNTVVQWDHYSFQIHGQRIFVFSGEFHYWRIPVPGLWRDILEKIKAAGFTAFAFYSSWAYHAPNNHTVDFSTGARDITPIFELAKELGLYIIVRPGPYVNAEANAGGFPLWLTTGEYGTLRNDDERYTAAWKPYFTKMSQITSKYQITDGENTLFYQIENEYGDQWIGDPSDRVPNNTAIAYMELLEASARENGINVPLTANDPNMNSKSWGKDWSNAGGNVDAPGLDSYPSCWTCDISQCTSTNGEYVPYKVMQYYDYFQEVQPTTPSFMPEFQGGSYNPWAGPEGGCSENTGADFANLFYRWNIGQHVTAMSLYMLYGGTNWGSLAAPVTASSYDYSAPISEDRSIGAKYYETKLLALFTRCARDLTMTELIGNGTQYTDNIAVEAYELRNPQTNAGFYVTIHSNSSSGTNEAFQLQVNTSVGGLTVPSHGGTIRLNGHQSKIIVTDFTFGSKTLLYSTAEVLTYAVLDDKPTLVLWVPTGESGEFSIKGVKSGSVSNCQGCSGMGFYQENGGLTVRFTQSSGMSILQLDDVRVVLLDRTSAYNFWAPALTNDPFVPETESVLIQGPYLVRGAKITESTLAVTGDSVDATSIEVFAPQTLDTITWNGKEVKTTRTEYGSLRASLAAPPSIKLPSLTSWKTKDSLPERLPSYDDSGEAWADANHMTTSNPHKPETYPVLYGDDYGFHNGIRLWRGYFNNTAKGVYLNIQGGTAFGWSAYLNGHFLSSYLGNATETQGNKTILFPSDILSTKPETNPNTLLIIHDDTGHDQTTGVLNPRGILEARLLDEDEKSSEDLAFTHWRVAGTAGGESNLDPVRGVYNEDGLYAERMGWHLPGFDDSDWSTINTTTSSTTSSPPLTFTNATIQFFRSVIPLDLPNNTDTSMSFILSTPSTSSKAYRAQIFINGYQYGRYNPHIGNQVVFPVPPGILDYHGDNTIGVAVWAQSEDGASIELDWRVNYVADSSLDVGRLDEGGSLRPGWSEERLRFA

SEQ ID NO: 77 - DNA, 3310 bp, Aspergillus lentulus
  sig_peptide 1..60
  mat_peptide 61..3307
  source 1..3310: mol_type = genomic DNA
  CDS 1..801
  CDS 851..1847
  CDS 1899..2192
  CDS 2246..2317
  CDS 2367..2454
  CDS 2518..3307
atggcgcacatctaccaacttctccttcttcttctttcaaatctgtggttcgcgacagctgctcagaaccagtcagagactgaatggcctcttcatgataatggcttgagcaaggtagtgcaatgggaccactatagcttccacgtcaacgggcagaggatcttcgtcttttccggcgaattccattactggcgtattccagtccccgagttgtggagggatgttctcgagaaggtgaaagctaccggtttcactgcgtttgcgttctactctagctgggcctatcatgcgcccaacaaccacacggtcgacttctcgaccggcgctcgcgatatcacgcccatctttgagcttgcaaaggagctcggcatgtatatgattgtgcgccccgggccctacgtcaatgctgaagccagcgcgggcggcttccctctgtggctgacgactggcgagtatggctcgctgcggaatgatgacccgcggtatacggccgcatggacgccgtactttgccaacatgtcgcaaatcactagcaagtatcaggttacggatggacataacacgctcgtctaccagattgagaatgagtacggtcagcagtggatcggagatcccaaggatcgcaagccgaataagactgcggttgcttacatggagctcttggaagcatctgctcgtgagaatggtatcactgtgccattgacaagcaacgatcccaacatgaactcgaaatcttggggatcggactggtccaatgctggaggcaatgtcgacgtggctggtttggattcttatccgtcggtgagttaccattagatcctttttatttgtttcgttctgactgttgaagtgctggacatgcgacgtgagccaatgtacctccaccaatggggagtatgttccctacaaagtgattgattattacgactacttccaagaagttcagccaactcttccctcgttcatgcccgagttccagggcggttcgtacaacccctgggccggtcctgaaggtggatgtcctcaggacaccggcgccgagtttgctaacctgttctaccgatggaacattggccagcgagtgaccgccatgagtctgtatatgctgtacggaggaaccaactggggtgcaattgctgctcctgtgacagcaaccagctacgactactccgctcccatctccgaagaccgctcgattggagccaagtattccgagaccaagctactggcattgttcacccgtaccgcaaaggacctcacaatgacagaggcgatcgggaacggaacacaatataccaccaacacagccgtccgtgcattcgagttgagaaatcctcagaccaacgccgggttctacgtcacattccacaacgacaccaccgttggtggaaatcaagcgttcaaactccatgtcaacacttctgtcggtgccttgactgtccccaagaacgagggtgtgatccagctgaatggtcatcaatccaagatcatcgtgaccgacttcacgctcggcaaacgtactcttctctattcaactgccgaggtcttgacctacgccgtttttgaagacaggcccaccctcgtgctctgggttcctactggggaatccggcgagttcgcgatcaagggagccaagtcaggaaaggttgaaaatggcgatggctgctcgggaatcaaatttgagagtgagaagaactatctcgtcgtgaatttctctcaggccaagggattgagcgtcttgcggctcgataatggtgtgcgcgtggttctgctcgacaaggccgccgcgtaccgcttctgggctcctgcattgacaaatgatcctgtcgtgcaagaggccgaaactggtaagttcacttcatgcgtagtacattgtcatttcatactaatggttacagtgctcgtccacggcccgtaccttgttcgctccgccagcgtgtcgaagtccacactggcgctccgaggagactcagtcgagaagacgacactggaaatcttcgcacctcacagcgtgagggagattacctggaatgggaaacaagtgaagacctctcagacttcatatggcagtctcaaagcgactctcgctgcaccgccgaccataaagttacccgctctcacctcctggagatccaacgacagcttgccggagcggcttccatcgtatgacgattccggaccggcctggattggtgagttggattccaatcgatctggcctggacgaaatctaatgcgtttgacagaggcaaaccacatgaccacatctaaccccagtaaacctgcaacccttccagtcctatacgcagacgaatacggtatgtcaacctctataccgacaccatcacaagtctaacccgcctacaggcttccacaacggcgtccgcctctggcgcggctacttcaacggctctgcttccggagtctacctcaacatccaaggaggaagcgccttgtacgttaccctccccatcccctctcaactatctcatcgaaactaacaacctcccctccgcagcggctggtccgcctggctaaacggccacttcctcgactcccacctcggcgacgcaacaacctcccaagcaaacaaaaccctccccttcccaccctccctcctcaaccccaccgaaaacgtcctcctcatcgtccacgacgacacaggccacgaccagacaaccggcgccctaaacccacgcggcatcctcgcggcccgcctcctctccaacgactcctcgtcccccgcgccggaattcacccgctggcgcctcgccggcaccgcaggcggggaatcgaacctcgatcccatccgcggcgtcttcaacgaggacggcctcttcgcagaacgcatgggctggcacctccccggcttcgacgacagcgcctggacggccgagaactcaactgcatccacctcggcactgagcttcaccggcgcaaccgtccgcttcttccgcaccgtcgtccccctcgatatccctgctggtctggacgtctccgtctccttcgtgctctcgaccccatcgaatgcgcccaagggataccgcgcacagctgttcgtcaatgggtaccagtatggtcggtacaacccacacatcggcaatcaggtggtgttccctgttccgccgggtattctcgattaccagggagataacacgatcgggttggcggtctgggcgcagacggaagagggggcgagtatccaggtggactggaaggtgaattacgtggcggatagctcgttgagtgtcgctggatttgggaaaggcttgaggccgggttggaccgaggagcggttgaagtttacctag

SEQ ID NO: 78 - protein, 1014 aa, Aspergillus lentulus
MAHIYQLLLLLLSNLWFATAAQNQSETEWPLHDNGLSKVVQWDHYSFHVNGQRIFVFSGEFHYWRIPVPELWRDVLEKVKATGFTAFAFYSSWAYHAPNNHTVDFSTGARDITPIFELAKELGMYMIVRPGPYVNAEASAGGFPLWLTTGEYGSLRNDDPRYTAAWTPYFANMSQITSKYQVTDGHNTLVYQIENEYGQQWIGDPKDRKPNKTAVAYMELLEASARENGITVPLTSNDPNMNSKSWGSDWSNAGGNVDVAGLDSYPSCWTCDVSQCTSTNGEYVPYKVIDYYDYFQEVQPTLPSFMPEFQGGSYNPWAGPEGGCPQDTGAEFANLFYRWNIGQRVTAMSLYMLYGGTNWGAIAAPVTATSYDYSAPISEDRSIGAKYSETKLLALFTRTAKDLTMTEAIGNGTQYTTNTAVRAFELRNPQTNAGFYVTFHNDTTVGGNQAFKLHVNTSVGALTVPKNEGVIQLNGHQSKIIVTDFTLGKRTLLYSTAEVLTYAVFEDRPTLVLWVPTGESGEFAIKGAKSGKVENGDGCSGIKFESEKNYLVVNFSQAKGLSVLRLDNGVRVVLLDKAAAYRFWAPALTNDPVVQEAETVLVHGPYLVRSASVSKSTLALRGDSVEKTTLEIFAPHSVREITWNGKQVKTSQTSYGSLKATLAAPPTIKLPALTSWRSNDSLPERLPSYDDSGPAWIEANHMTTSNPSKPATLPVLYADEYGFHNGVRLWRGYFNGSASGVYLNIQGGSAFGWSAWLNGHFLDSHLGDATTSQANKTLPFPPSLLNPTENVLLIVHDDTGHDQTTGALNPRGILAARLLSNDSSSPAPEFTRWRLAGTAGGESNLDPIRGVFNEDGLFAERMGWHLPGFDDSAWTAENSTASTSALSFTGATVRFFRTVVPLDIPAGLDVSVSFVLSTPSNAPKGYRAQLFVNGYQYGRYNPHIGNQVVFPVPPGILDYQGDNTIGLAVWAQTEEGASIQVDWKVNYVADSSLSVAGFGKGLRPGWTEERLKFT

SEQ ID NO: 79 - protein, 994 aa, Aspergillus lentulus
  REGION 1..994: note = mat_peptide
AQNQSETEWPLHDNGLSKVVQWDHYSFHVNGQRIFVFSGEFHYWRIPVPELWRDVLEKVKATGFTAFAFYSSWAYHAPNNHTVDFSTGARDITPIFELAKELGMYMIVRPGPYVNAEASAGGFPLWLTTGEYGSLRNDDPRYTAAWTPYFANMSQITSKYQVTDGHNTLVYQIENEYGQQWIGDPKDRKPNKTAVAYMELLEASARENGITVPLTSNDPNMNSKSWGSDWSNAGGNVDVAGLDSYPSCWTCDVSQCTSTNGEYVPYKVIDYYDYFQEVQPTLPSFMPEFQGGSYNPWAGPEGGCPQDTGAEFANLFYRWNIGQRVTAMSLYMLYGGTNWGAIAAPVTATSYDYSAPISEDRSIGAKYSETKLLALFTRTAKDLTMTEAIGNGTQYTTNTAVRAFELRNPQTNAGFYVTFHNDTTVGGNQAFKLHVNTSVGALTVPKNEGVIQLNGHQSKIIVTDFTLGKRTLLYSTAEVLTYAVFEDRPTLVLWVPTGESGEFAIKGAKSGKVENGDGCSGIKFESEKNYLVVNFSQAKGLSVLRLDNGVRVVLLDKAAAYRFWAPALTNDPVVQEAETVLVHGPYLVRSASVSKSTLALRGDSVEKTTLEIFAPHSVREITWNGKQVKTSQTSYGSLKATLAAPPTIKLPALTSWRSNDSLPERLPSYDDSGPAWIEANHMTTSNPSKPATLPVLYADEYGFHNGVRLWRGYFNGSASGVYLNIQGGSAFGWSAWLNGHFLDSHLGDATTSQANKTLPFPPSLLNPTENVLLIVHDDTGHDQTTGALNPRGILAARLLSNDSSSPAPEFTRWRLAGTAGGESNLDPIRGVFNEDGLFAERMGWHLPGFDDSAWTAENSTASTSALSFTGATVRFFRTVVPLDIPAGLDVSVSFVLSTPSNAPKGYRAQLFVNGYQYGRYNPHIGNQVVFPVPPGILDYQGDNTIGLAVWAQTEEGASIQVDWKVNYVADSSLSVAGFGKGLRPGWTEERLKFT

SEQ ID NO: 80 - skipped

SEQ ID NO: 81 - protein, 6 aa, synthetic construct
  REGION 1..6: note = SEQ ID NO: 81 is the conserved motif K[Y/F][Y/S]ETK.
  SITE 2: note = MISC_FEATURE - The amino acid in position 2 of the conserved motif is either phenylalanine (F) or tyrosine (Y).
  SITE 3: note = MISC_FEATURE - The amino acid in position 3 of the conserved motif is either serine (S) or tyrosine (Y).
KXXETK

SEQ ID NO: 82 - protein, 1013 aa, Penicillium chrysogenum
MTRILNCLLVLLACLGVSSKAEDQAVTQWPLQDNGLNTVVQWDHYSFQINGQRIFIFSGEFHYWRIPVPALWRDILEKIKAAGFTAFAFYSSWAYHAPNNATVDFTTGARDITPIFELAKELGMYIIVRPGPYVNAEANAGGFPLWVTTGDYGTLRNDDTRYTNAWTPYFTEVTEITSRYQVTDGHYSIVYQIENEYGNQWLGDPTLRVPNETAIAYMELLKANARDNGITLPLTVNDPNMKTHSWGKDWSDAGGNVDAAGLDSYPSCWTCDISQCTSTNGAYVPFQVLEYHDYFQESQPSMPAFMPEFQGGSYNPWGGPEGGCPGDIGDDFANLFYRWNIGQRVTAMSLYMMFGGQNPGAMAAPVTASSYDYSAPISEDRSIWSKYHETKLLALFTRSAKDLTMTELMGNGTQYTDNPAVRAYELRNPETNSAFYATFHSNTSISTNEPFHLKVNTSAGVLTVPKYASTIRLNGHQSKIIVTDFTFGSKSLLYSTAEVLTYAVFDKKPTLVLWVPTGESGEFSIKGAKKGSIKKCQGCSRVKFIKEHGGLTTSLTQSAGMTVLEFDDGVRVILLDRTSAYDFWAPALTNDPFVPETESVLIQGPYLVRDAKLSGSKLAITGDVVNATTLDVFAPKGVKSVTWNGKKVDTHSTEYGSLKGSLDAPQSIKLPALASWKSKDSLPERFADYDDSGAAWVDANHMTTLNPRTPTSLPVLYADQYGFHNGVRLWRGYFNGTATGAFINVQGGSAFGWSAWLNGEFLASHLGNATTSQANLSLSFTDATLHTDTPNVLLIVHDDTGHDQTTGALNPRGIMDAKLLGSDSGFTHWRLAGTAGGESDLDPVRGVYNEDGLFAERVGWHLPGFDDSDWGEEASAKDSTTSVLSFEGATVRFFRTTCPLDIPAHTDVSISFVLSTPAGATTEYRAQLFVNGYQYGRYNPYIGNQVVYPVPVGILDYKGENTIGVAVWAQSEEGASIGIDWRVNYLADSSLDVASWDTKDLRPGWTEERVKYA

SEQ ID NO: 83 - protein, 352 aa, Penicillium chrysogenum
MLPHLLLAAAQLFASSSAALTYNGADISSLLVEEGKGVSYKNLAGTPEKLETILSASGVNSVRQRIWVNPSDGSYDLDYNVKLAKRVQAQGMGTYLDLHYSDTWADPKSQTTPSGWSTTDIGILAGQVYDYTLDVCNTFAANKIDVDIVSIGNEIRNGLLWPLGGTSNYNNIARLLHSAAWGVKDSKLATTPKIMIHLDNGWDSGAQSYFYDQVLAPGSGLVSTDFDYIGVSYYPFYNADATLAALKTSLTNLHSKYKKETLVVETNWPFSCPNPEYAFPTDLKDIPFSVEGQQTFLQRLAKAVEEVGGLGIYYWEPAWVDNAGLGSSCDDNLFFAWSNDQARASLDTLGGL

SEQ ID NO: 84 - protein, 1007 aa, Aspergillus niger
MKLSSACAIALLAAQAAGASIKHRINGFTLTEHSDPAKRELLQKYVTWDDKSLFINGERIMIFSGEFHPFRLPVKELQLDIFQKVKALGFNCVSFYVDWALVEGKPGEYRADGIFDLEPFFDAASEAGIYLLARPGPYINAESSGGGFPGWLQRVNGTLRSSDKAYLDATDNYVSHVAATIAKYQITNGGPIILYQPENEYTSGCCGVEFPDPVYMQYVEDQARNAGVVIPLINNDASASGNNAPGTGKGAVDIYGHDSYPLGFDCANPTVWPSGDLPTNFRTLHLEQSPTTPYAIVEFQGGSYDPWGGPGFAACSELLNNEFERVFYKNDFSFQIAIMNLYMIFGGTNWGNLGYPNGYTSYDYGSAVTESRNITREKYSELKLLGNFAKVSPGYLTASPGNLTTSGYADTTDLTVTPLLGNSTGSFFVVRHSDYSSEESTSYKLRLPTSAGSVTIPQLGGTLTLNGRDSKIHVTDYNVSGTNIIYSTAEVFTWKKFADGKVLVLYGGAGEHHELAISTKSNVTVIEGSESGISSKQTSSSVVVGWDVSTTRRIIQVGDLKILLLDRNSAYNYWVPQLATDGTSPGFSTPEKVASSIIVKAGYLVRTAYLKGSGLYLTADFNATTSVEVIGVPSTAKNLFINGDKTSHTVDKNGIWSATVDYNAPDISLPSLKDLDWKYVDTLPEIQSSYDDSLWPAADLKQTKNTLRSLTTPTSLYSSDYGFHTGYLLYRGHFTATGNESTFAIDTQGGSAFGSSVWLNGTYLGSWTGLYANSDYNATYNLPQLQAGKTYVITVVIDNMGLEENWTVGEDLMKTPRGILNFLLAGRPSSAISWKLTGNLGGEDYEDKVRGPLNEGGLYAERQGFHQPEPPSQNWKSSSPLEGLSEAGIGFYSASFDLDLPKGWDVPLFLNIGNSTTPSPYRVQVYVNGYQYAKYISNIGPQTSFPVPEGILNYRGTNWLAVTLWALDSAGGKLESLELSYTTPVLTALGEVESVDQPKYKKRKGAY

SEQ ID NO: 85 - protein, 350 aa, Aspergillus niger
MIYPLLLSALPLLSSAALTYRGADISSLLIEEDAGISYKNLNGETQALEDILVNNGVNSIRQRVWVDPSDGSYDLDYNLKLAKRVQAAGMSIYLDLHLSDTWADPSDQTTPTGWSTTDIDTLTWQLYNYTLDVCNTFAENDIDIEIVSIGNEISSGLLWPLGKTSNYDNIAKLLHSGAWGVKDSNQATTPKIMIHLDNGWDWEEQEYFYKTVLATGSLLSTDFDLMGVSYYPFYNSEATLSALQTSLTNMQSNYDKSVVVVETNWPVSCPDPEYSFPSDLSSIPFSAAGQEEFLEKLAEVVEGVTDGLGIYYWEPAWVDNAALASSCADNLMVDIDTDEVLESVTVFEDL